European Patent Specification EP 4 259 796 B1, published September 3, 2025. Title: Therapeutics for the treatment of neurodegenerative disorders. Applicant: UCL Business Ltd THE UNITED STATES OF AMERICA, AS REPRESENTED BY THE SECRETARY, DEPARTMENT OF HEALTH AND HUMAN SERVICES. The sequence listing filed with the application follows.

SEQUENCE LISTING (580 sequences)

SEQ ID NO: 1 - RNA, 1288 nt, Homo sapiens
  misc_feature (414)..(414): G can be replaced with C at this position
  misc_feature (964)..(964): U can be replaced with G at this position
gugagggucauugcucggccccucccaugccacuuccacucaccauuccugccugcccagcucuuccucuuucuggccacaccauccacacucuccuggcccucugagacugcccgccaugccauucccuuuaccuggaaaacuccucccuauccaucaaaguccagauucagggucaccuccucugggaagcccaccuuggccuccagguugacucucacuacucaucaucagguucuuccuucuauuccagcccuaaccacucaggauugggccguuugugucuggguaugucucuuccagcugccuggguuuccuggaaagaacucuuauccccaggaacuaguuuguugaauaaaugcuggugaaugaaugaaugauugaacagaugaaugagugaugaguagauaaaaggauggauggagagaugggugaguacauggauggauagauggaugaguugguggguagauucguggcuagauggaugauggauggauggacagauggauggauauaugauugaacuauugaaaguauagauguauggaugggugaauuuggggguaauuguuagaugauggaugaguauagaugaaugauggauggauaacuugaugaguggauagauagauugcuggauagaugauugacuggguggauagaugaaauguuggaugagcagauuaaguuguauuggaugggauggauggaagugugguugaguuauuagaaggaagauugaguagauaggugaauuuguugauagucagauggguagauagguagauggauggauggauggauggauguauaggcagauggacaaauggaugaauggguggguggaugaauggaaggaugugugguugaacuauugcaaguauugauaauuggguucauaauuucugaauauuuagauggaugguugugaguggcugguggacagacgaaaaauggaugguuggauaaauugauggguggauggaugguugguuguaugaaagaaugaaugauuggguagguggauuaaguugcggaucaauguaugggauggaugaauggauggauggauggaugugugguugaauuacugaaagguuggaagaguggaugggugaaauuugggguaguuagauggguggguguguggauggauaaaagaguagaugaaugaauuaaugaauaaacaggcagauggaugauguaagcugccccagacccugggaccucugacccccggcgaccccuugcacucuccaugacacuuucucucccaugguggcag

SEQ ID NO: 2 - RNA, 128 nt, Homo sapiens
  misc_feature (112)..(112): G can be replaced with C at this position
cugccuggguuuccuggaaagaacucuuauccccaggaacuaguuuguugaauaaaugcuggugaaugaaugaaugauugaacagaugaaugagugaugaguagauaaaaggauggauggagagaugg

SEQ ID NO: 3 - RNA, 178 nt, Homo sapiens
  misc_feature (162)..(162): G at this position can be replaced with C
cccuaaccacucaggauugggccguuugugucuggguaugucucuuccagcugccuggguuuccuggaaagaacucuuauccccaggaacuaguuuguugaauaaaugcuggugaaugaaugaaugauugaacagaugaaugagugaugaguagauaaaaggauggauggagagaugg

SEQ ID NO: 4 - RNA, 13 nt, Artificial Sequence
  SEQ ID NO:4
  misc_feature (1)..(13): U can be replaced with T
  misc_feature (1)..(13): U can be replaced by T. Any base can be replaced with a modified base.
ggaguuuuccagg

SEQ ID NO: 5 - RNA, 13 nt, Artificial Sequence
  SEQ ID NO 5
  misc_feature: U can be replaced by T. Any base can be replaced with a modified base.
aggaguuuuccag

SEQ ID NO: 6 - RNA, 13 nt, Artificial Sequence
  SEQ ID NO 6
  misc_feature (1)..(13): U can be replaced by T. Any base can be replaced with a modified base.
gaggaguuuucca

SEQ ID NO: 7 - RNA, 13 nt, Artificial Sequence
  SEQ ID NO 7
  misc_feature (1)..(13): U can be replaced by T. Any base can be replaced with a modified base.
ggaggaguuuucc

SEQ ID NO: 8 - RNA, 13 nt, Artificial Sequence
  GGGAGGAGUUUUC
  misc_feature (1)..(13): U can be replaced by T. Any base can be replaced with a modified base.
gggaggaguuuuc

SEQ ID NO: 9 - RNA, 13 nt, Artificial Sequence
  SEQ ID NO 9
  misc_feature (1)..(13): U can be replaced by T. Any base can be replaced with a modified base.
agggaggaguuuu

SEQ ID NO: 10 - RNA, 13 nt, Artificial Sequence
  SEQ ID NO 10
  misc_feature (1)..(13): U can be replaced by T. Any base can be replaced with a modified base.
uagggaggaguuu

SEQ ID NO: 11 - RNA, 13 nt, Artificial Sequence
  SEQ ID NO 11
  misc_feature (1)..(13): U can be replaced by T. Any base can be replaced with a modified base.
auagggaggaguu

SEQ ID NO: 12 - RNA, 13 nt, Artificial Sequence
  SEQ ID NO 12
  misc_feature (1)..(13): U can be replaced by T. Any base can be replaced with a modified base.
gauagggaggagu

SEQ ID NO: 13 - RNA, 13 nt, Artificial Sequence
  SEQ ID NO 13
  misc_feature (1)..(13): U can be replaced by T. Any base can be replaced with a modified base.
ggauagggaggag

SEQ ID NO: 14 - RNA, 13 nt, Artificial Sequence
  SEQ ID NO 14
  misc_feature (1)..(13): U can be replaced by T. Any base can be replaced with a modified base.
uggauagggagga

SEQ ID NO: 15 - RNA, 13 nt, Artificial Sequence
  SEQ ID NO 15
  misc_feature (1)..(13): U can be replaced by T. Any base can be replaced with a modified base.
auggauagggagg

SEQ ID NO: 16 - RNA, 13 nt, Artificial Sequence
  SEQ ID NO 16
  misc_feature (1)..(13): U can be replaced by T. Any base can be replaced with a modified base.
gauggauagggag

SEQ ID NO: 17 - RNA, 13 nt, Artificial Sequence
  SEQ ID NO 17
  misc_feature (1)..(13): U can be replaced by T. Any base can be replaced with a modified base.
ugauggauaggga

SEQ ID NO: 18 - RNA, 13 nt, Artificial Sequence
  SEQ ID NO 18
  misc_feature (1)..(13): U can be replaced by T. Any base can be replaced with a modified base.
uugauggauaggg

SEQ ID NO: 19 - RNA, 13 nt, Artificial Sequence
  SEQ ID NO 19
  misc_feature (1)..(13): U can be replaced by T. Any base can be replaced with a modified base.
uuugauggauagg

SEQ ID NO: 20 - RNA, 13 nt, Artificial Sequence
  SEQ ID NO 20
  misc_feature (1)..(13): U can be replaced by T. Any base can be replaced with a modified base.
cuuugauggauag

SEQ ID NO: 21 - RNA, 13 nt, Artificial Sequence
  SEQ ID NO 21
  misc_feature (1)..(13): U can be replaced by T. Any base can be replaced with a modified base.
acuuugauggaua

SEQ ID NO: 22 - RNA, 13 nt, Artificial Sequence
  SEQ ID NO 22
  misc_feature (1)..(13): U can be replaced by T. Any base can be replaced with a modified base.
gacuuugauggau

SEQ ID NO: 23 - RNA, 13 nt, Artificial Sequence
  SEQ ID NO 23
  misc_feature (1)..(13): U can be replaced by T. Any base can be replaced with a modified base.
ggacuuugaugga

SEQ ID NO: 24 - RNA, 13 nt, Artificial Sequence
  SEQ ID NO 24
  misc_feature (1)..(13): U can be replaced by T. Any base can be replaced with a modified base.
uggacuuugaugg

SEQ ID NO: 25 - RNA, 13 nt, Artificial Sequence
  SEQ ID NO 25
  misc_feature (1)..(13): U can be replaced by T. Any base can be replaced with a modified base.
cuggacuuugaug

SEQ ID NO: 26 - RNA, 13 nt, Artificial Sequence
  SEQ ID NO 26
  misc_feature (1)..(13): U can be replaced by T. Any base can be replaced with a modified base.
ucuggacuuugau

SEQ ID NO: 27 - RNA, 13 nt, Artificial Sequence
  SEQ ID NO 27
  misc_feature (1)..(13): U can be replaced by T. Any base can be replaced with a modified base.
aucuggacuuuga

SEQ ID NO: 28 - RNA, 13 nt, Artificial Sequence
  SEQ ID NO 28
  misc_feature (1)..(13): U can be replaced by T. Any base can be replaced with a modified base.
aaucuggacuuug

SEQ ID NO: 29 - RNA, 13 nt, Artificial Sequence
  SEQ ID NO 29
  misc_feature (1)..(13): U can be replaced by T. Any base can be replaced with a modified base.
gaaucuggacuuu

SEQ ID NO: 30 - RNA, 13 nt, Artificial Sequence
  UGAAUCUGGACUU
  misc_feature (1)..(13): U can be replaced by T. Any base can be replaced with a modified base.
ugaaucuggacuu

SEQ ID NO: 31 - RNA, 13 nt, Artificial Sequence
  SEQ ID NO 31
  misc_feature (1)..(13): U can be replaced by T. Any base can be replaced with a modified base.
cugaaucuggacu

SEQ ID NO: 32 - RNA, 13 nt, Artificial Sequence
  SEQ ID NO 32
  misc_feature (1)..(13): U can be replaced by T. Any base can be replaced with a modified base.
ccugaaucuggac

SEQ ID NO: 33 - RNA, 13 nt, Artificial Sequence
  SEQ ID NO 33
  misc_feature (1)..(13): U can be replaced by T. Any base can be replaced with a modified base.
cccugaaucugga

SEQ ID NO: 34 - RNA, 13 nt, Artificial Sequence
  SEQ ID NO 34
  misc_feature (1)..(13): U can be replaced by T. Any base can be replaced with a modified base.
acccugaaucugg

SEQ ID NO: 35 - RNA, 13 nt, Artificial Sequence
  SEQ ID NO 35
  misc_feature (1)..(13): U can be replaced by T. Any base can be replaced with a modified base.
gacccugaaucug

SEQ ID NO: 36 - RNA, 13 nt, Artificial Sequence
  SEQ ID NO 36
  misc_feature (1)..(13): U can be replaced by T. Any base can be replaced with a modified base.
ugacccugaaucu

SEQ ID NO: 37 - RNA, 13 nt, Artificial Sequence
  GUGACCCUGAAUC
  misc_feature (1)..(13): U can be replaced by T. Any base can be replaced with a modified base.
gugacccugaauc

SEQ ID NO: 38 - RNA, 13 nt, Artificial Sequence
  GGUGACCCUGAAU
  misc_feature (1)..(13): U can be replaced by T. Any base can be replaced with a modified base.
ggugacccugaau

SEQ ID NO: 39 - RNA, 13 nt, Artificial Sequence
  SEQ ID NO 39
  misc_feature (1)..(13): U can be replaced by T. Any base can be replaced with a modified base.
aggugacccugaa

SEQ ID NO: 40 - RNA, 13 nt, Artificial Sequence
  SEQ ID NO 40
  misc_feature (1)..(13): U can be replaced by T. Any base can be replaced with a modified base.
gaggugacccuga

SEQ ID NO: 41 - RNA, 13 nt, Artificial Sequence
  SEQ ID NO 41
  misc_feature (1)..(13): U can be replaced by T. Any base can be replaced with a modified base.
ggaggugacccug

SEQ ID NO: 42 - RNA, 13 nt, Artificial Sequence
  SEQ ID NO 42
  misc_feature (1)..(13): U can be replaced by T. Any base can be replaced with a modified base.
aggaggugacccu

SEQ ID NO: 43 - RNA, 13 nt, Artificial Sequence
  SEQ ID NO 43
  misc_feature (1)..(13): U can be replaced by T. Any base can be replaced with a modified base.
gaggaggugaccc

SEQ ID NO: 44 - RNA, 13 nt, Artificial Sequence
  SEQ ID NO 44
  misc_feature (1)..(13): U can be replaced by T. Any base can be replaced with a modified base.
agaggaggugacc

SEQ ID NO: 45 - RNA, 13 nt, Artificial Sequence
  SEQ ID NO 45
  misc_feature (1)..(13): U can be replaced by T. Any base can be replaced with a modified base.
cagaggaggugac

SEQ ID NO: 46 - RNA, 13 nt, Artificial Sequence
  SEQ ID NO 46
  misc_feature (1)..(13): U can be replaced by T. Any base can be replaced with a modified base.
ccagaggagguga

SEQ ID NO: 47 - RNA, 13 nt, Artificial Sequence
  SEQ ID NO 47
  misc_feature (1)..(13): U can be replaced by T. Any base can be replaced with a modified base.
cccagaggaggug

SEQ ID NO: 48 - RNA, 13 nt, Artificial Sequence
  SEQ ID NO 48
  misc_feature (1)..(13): U can be replaced by T. Any base can be replaced with a modified base.
ucccagaggaggu

SEQ ID NO: 49 - RNA, 13 nt, Artificial Sequence
  SEQ ID NO 49
  misc_feature (1)..(13): U can be replaced by T. Any base can be replaced with a modified base.
uucccagaggagg

SEQ ID NO: 50 - RNA, 13 nt, Artificial Sequence
  SEQ ID NO 50
  misc_feature (1)..(13): U can be replaced by T. Any base can be replaced with a modified base.
cuucccagaggag

SEQ ID NO: 51 - RNA, 13 nt, Artificial Sequence
  SEQ ID NO 51
  misc_feature (1)..(13): U can be replaced by T. Any base can be replaced with a modified base.
gcuucccagagga

SEQ ID NO: 52 - RNA, 13 nt, Artificial Sequence
  SEQ ID NO 52
  misc_feature (1)..(13): U can be replaced by T. Any base can be replaced with a modified base.
ggcuucccagagg

SEQ ID NO: 53 - RNA, 13 nt, Artificial Sequence
  SEQ ID NO 53
  misc_feature (1)..(13): U can be replaced by T. Any base can be replaced with a modified base.
gggcuucccagag

SEQ ID NO: 54 - RNA, 13 nt, Artificial Sequence
  UGGGCUUCCCAGA
  misc_feature (1)..(13): U can be replaced by T. Any base can be replaced with a modified base.
ugggcuucccaga

SEQ ID NO: 55 - RNA, 13 nt, Artificial Sequence
  SEQ ID NO 55
  misc_feature (1)..(13): U can be replaced by T. Any base can be replaced with a modified base.
gugggcuucccag

SEQ ID NO: 56 - RNA, 13 nt, Artificial Sequence
  SEQ ID NO 56
  misc_feature (1)..(13): U can be replaced by T. Any base can be replaced with a modified base.
ggugggcuuccca

SEQ ID NO: 57 - RNA, 13 nt, Artificial Sequence
  SEQ ID NO 57
  misc_feature (1)..(13): U can be replaced by T. Any base can be replaced with a modified base.
aggugggcuuccc

SEQ ID NO: 58 - RNA, 13 nt, Artificial Sequence
  SEQ ID NO 58
  misc_feature (1)..(13): U can be replaced by T. Any base can be replaced with a modified base.
aaggugggcuucc

SEQ ID NO: 59 - RNA, 13 nt, Artificial Sequence
  SEQ ID NO 59
  misc_feature (1)..(13): U can be replaced by T. Any base can be replaced with a modified base.
caaggugggcuuc

SEQ ID NO: 60 - RNA, 13 nt, Artificial Sequence
  SEQ ID NO 60
  misc_feature (1)..(13): U can be replaced by T. Any base can be replaced with a modified base.
ccaaggugggcuu

SEQ ID NO: 61 - RNA, 13 nt, Artificial Sequence
  SEQ ID NO 61
  misc_feature (1)..(13): U can be replaced by T. Any base can be replaced with a modified base.
gccaaggugggcu

SEQ ID NO: 62 - RNA, 13 nt, Artificial Sequence
  SEQ ID NO 62
  misc_feature (1)..(13): U can be replaced by T. Any base can be replaced with a modified base.
ggccaaggugggc

SEQ ID NO: 63 - RNA, 13 nt, Artificial Sequence
  SEQ ID NO 63
  misc_feature (1)..(13): U can be replaced by T. Any base can be replaced with a modified base.
aggccaagguggg

SEQ ID NO: 64 - RNA, 13 nt, Artificial Sequence
  SEQ ID NO 64
  misc_feature (1)..(13): U can be replaced by T. Any base can be replaced with a modified base.
gaggccaaggugg

SEQ ID NO: 65 - RNA, 13 nt, Artificial Sequence
  SEQ ID NO 65
  misc_feature (1)..(13): U can be replaced by T. Any base can be replaced with a modified base.
ggaggccaaggug

SEQ ID NO: 66 - RNA, 13 nt, Artificial Sequence
  SEQ ID NO 66
  misc_feature (1)..(13): U can be replaced by T. Any base can be replaced with a modified base.
uggaggccaaggu

SEQ ID NO: 67 - RNA, 13 nt, Artificial Sequence
  SEQ ID NO 67
  misc_feature (1)..(13): U can be replaced by T. Any base can be replaced with a modified base.
cuggaggccaagg

SEQ ID NO: 68 - RNA, 13 nt, Artificial Sequence
  SEQ ID NO 68
  misc_feature (1)..(13): U can be replaced by T. Any base can be replaced with a modified base.
ccuggaggccaag

SEQ ID NO: 69 - RNA, 13 nt, Artificial Sequence
  SEQ ID NO 69
  misc_feature (1)..(13): U can be replaced by T. Any base can be replaced with a modified base.
accuggaggccaa

SEQ ID NO: 70 - RNA, 13 nt, Artificial Sequence
  SEQ ID NO 70
  misc_feature (1)..(13): U can be replaced by T. Any base can be replaced with a modified base.
aaccuggaggcca

SEQ ID NO: 71 - RNA, 13 nt, Artificial Sequence
  SEQ ID NO 71
  misc_feature (1)..(13): U can be replaced by T. Any base can be replaced with a modified base.
caaccuggaggcc

SEQ ID NO: 72 - RNA, 13 nt, Artificial Sequence
  SEQ ID NO 72
  misc_feature (1)..(13): U can be replaced by T. Any base can be replaced with a modified base.
ucaaccuggaggc

SEQ ID NO: 73 - RNA, 13 nt, Artificial Sequence
  SEQ ID NO 73
  misc_feature (1)..(13): U can be replaced by T. Any base can be replaced with a modified base.
gucaaccuggagg

SEQ ID NO: 74 - RNA, 13 nt, Artificial Sequence
  SEQ ID NO 74
  misc_feature (1)..(13): U can be replaced by T. Any base can be replaced with a modified base.
agucaaccuggag

SEQ ID NO: 75 - RNA, 13 nt, Artificial Sequence
  SEQ ID NO 75
  misc_feature (1)..(13): U can be replaced by T. Any base can be replaced with a modified base.
gagucaaccugga

SEQ ID NO: 76 - RNA, 13 nt, Artificial Sequence
  SEQ ID NO 76
  misc_feature (1)..(13): U can be replaced by T. Any base can be replaced with a modified base.
agagucaaccugg

SEQ ID NO: 77 - RNA, 13 nt, Artificial Sequence
  SEQ ID NO 77
  misc_feature (1)..(13): U can be replaced by T. Any base can be replaced with a modified base.
gagagucaaccug

SEQ ID NO: 78 - RNA, 13 nt, Artificial Sequence
  SEQ ID NO 78
  misc_feature (1)..(13): U can be replaced by T. Any base can be replaced with a modified base.
ugagagucaaccu

SEQ ID NO: 79 - RNA, 13 nt, Artificial Sequence
  SEQ ID NO 79
  misc_feature (1)..(13): U can be replaced by T. Any base can be replaced with a modified base.
gugagagucaacc

SEQ ID NO: 80 - RNA, 13 nt, Artificial Sequence
  SEQ ID NO 80
  misc_feature (1)..(13): U can be replaced by T. Any base can be replaced with a modified base.
agugagagucaac

SEQ ID NO: 81 - RNA, 13 nt, Artificial Sequence
  SEQ ID NO 81
  misc_feature (1)..(13): U can be replaced by T. Any base can be replaced with a modified base.
uagugagagucaa

SEQ ID NO: 82 - RNA, 13 nt, Artificial Sequence
  SEQ ID NO 82
  misc_feature (1)..(13): U can be replaced by T. Any base can be replaced with a modified base.
guagugagaguca

SEQ ID NO: 83 - RNA, 13 nt, Artificial Sequence
  SEQ ID NO 83
  misc_feature (1)..(13): U can be replaced by T. Any base can be replaced with a modified base.
aguagugagaguc

SEQ ID NO: 84 - RNA, 13 nt, Artificial Sequence
  SEQ ID NO 84
  misc_feature: U can be replaced by T. Any base can be replaced with a modified base.
gaguagugagagu

SEQ ID NO: 85 - RNA, 13 nt, Artificial Sequence
  SEQ ID NO 85
  misc_feature (1)..(13): U can be replaced by T. Any base can be replaced with a modified base.
ugaguagugagag

SEQ ID NO: 86 - RNA, 13 nt, Artificial Sequence
  SEQ ID NO 86
  misc_feature (1)..(13): U can be replaced by T. Any base can be replaced with a modified base.
augaguagugaga

SEQ ID NO: 87 - RNA, 13 nt, Artificial Sequence
  SEQ ID NO 88
  misc_feature (1)..(13): U can be replaced by T. Any base can be replaced with a modified base.
gaugaguagugag

SEQ ID NO: 88 - RNA, 13 nt, Artificial Sequence
  SEQ ID NO 88
  misc_feature (1)..(13): U can be replaced by T. Any base can be replaced with a modified base.
ugaugaguaguga

SEQ ID NO: 89 - RNA, 13 nt, Artificial Sequence
  SEQ ID NO 89
  misc_feature (1)..(13): U can be replaced by T. Any base can be replaced with a modified base.
augaugaguagug

SEQ ID NO: 90 - RNA, 13 nt, Artificial Sequence
  SEQ ID NO 90
  misc_feature (1)..(13): U can be replaced by T. Any base can be replaced with a modified base.
gaugaugaguagu

SEQ ID NO: 91 - RNA, 13 nt, Artificial Sequence
  SEQ ID NO 91
  misc_feature (1)..(13): U can be replaced by T. Any base can be replaced with a modified base.
ugaugaugaguag

SEQ ID NO: 92 - RNA, 13 nt, Artificial Sequence
  SEQ ID NO 92
  misc_feature (1)..(13): U can be replaced by T. Any base can be replaced with a modified base.
cugaugaugagua

SEQ ID NO: 93 - RNA, 13 nt, Artificial Sequence
  SEQ ID NO 93
  misc_feature (1)..(13): U can be replaced by T. Any base can be replaced with a modified base.
ccugaugaugagu

SEQ ID NO: 94 - RNA, 13 nt, Artificial Sequence
  SEQ ID NO 94
  misc_feature (1)..(13): U can be replaced by T. Any base can be replaced with a modified base.
accugaugaugag

SEQ ID NO: 95 - RNA, 13 nt, Artificial Sequence
  SEQ ID NO 95
  misc_feature (1)..(13): U can be replaced by T. Any base can be replaced with a modified base.
aaccugaugauga

SEQ ID NO: 96 - RNA, 13 nt, Artificial Sequence
  SEQ ID NO 96
  misc_feature (1)..(13): U can be replaced by T. Any base can be replaced with a modified base.
gaaccugaugaug

SEQ ID NO: 97 - RNA, 13 nt, Artificial Sequence
  SEQ ID NO 97
  misc_feature (1)..(13): U can be replaced by T. Any base can be replaced with a modified base.
agaaccugaugau

SEQ ID NO: 98 - RNA, 13 nt, Artificial Sequence
  SEQ ID NO 99
  misc_feature (1)..(13): U can be replaced by T. Any base can be replaced with a modified base.
aagaaccugauga

SEQ ID NO: 99 - RNA, 13 nt, Artificial Sequence
  SEQ ID NO 99
  misc_feature (1)..(13): U can be replaced by T. Any base can be replaced with a modified base.
gaagaaccugaug

SEQ ID NO: 100 - RNA, 13 nt, Artificial Sequence
  SEQ ID NO 100
  misc_feature (1)..(13): U can be replaced by T. Any base can be replaced with a modified base.
ggaagaaccugau

SEQ ID NO: 101 - RNA, 13 nt, Artificial Sequence
  SEQ ID NO 101
  misc_feature (1)..(13): U can be replaced by T. Any base can be replaced with a modified base.
aggaagaaccuga

SEQ ID NO: 102 - RNA, 13 nt, Artificial Sequence
  SEQ ID NO 102
  misc_feature (1)..(13): U can be replaced by T. Any base can be replaced with a modified base.
aaggaagaaccug

SEQ ID NO: 103 - RNA, 13 nt, Artificial Sequence
  SEQ ID NO 103
  misc_feature (1)..(13): U can be replaced by T. Any base can be replaced with a modified base.
gaaggaagaaccu

SEQ ID NO: 104 - RNA, 13 nt, Artificial Sequence
  SEQ ID NO 104
  misc_feature (1)..(13): U can be replaced by T. Any base can be replaced with a modified base.
agaaggaagaacc

SEQ ID NO: 105 - RNA, 13 nt, Artificial Sequence
  SEQ ID NO 105
  misc_feature (1)..(13): U can be replaced by T. Any base can be replaced with a modified base.
uagaaggaagaac

SEQ ID NO: 106 - RNA, 13 nt, Artificial Sequence
  SEQ ID NO 106
  misc_feature (1)..(13): U can be replaced by T. Any base can be replaced with a modified base.
auagaaggaagaa

SEQ ID NO: 107 - RNA, 13 nt, Artificial Sequence
  SEQ ID NO 107
  misc_feature (1)..(13): U can be replaced by T. Any base can be replaced with a modified base.
aauagaaggaaga

SEQ ID NO: 108 - RNA, 13 nt, Artificial Sequence
  GAAUAGAAGGAAG
  misc_feature (1)..(13): U can be replaced by T. Any base can be replaced with a modified base.
gaauagaaggaag

SEQ ID NO: 109 - RNA, 13 nt, Artificial Sequence
  SEQ ID NO 109
  misc_feature (1)..(13): U can be replaced by T. Any base can be replaced with a modified base.
ggaauagaaggaa

SEQ ID NO: 110 - RNA, 13 nt, Artificial Sequence
  SEQ ID NO 110
  misc_feature (1)..(13): U can be replaced by T. Any base can be replaced with a modified base.
uggaauagaagga

SEQ ID NO: 111 - RNA, 13 nt, Artificial Sequence
  SEQ ID NO 111
  misc_feature (1)..(13): U can be replaced by T. Any base can be replaced with a modified base.
cuggaauagaagg

SEQ ID NO: 112 - RNA, 13 nt, Artificial Sequence
  SEQ ID NO 112
  misc_feature (1)..(13): U can be replaced by T. Any base can be replaced with a modified base.
gcuggaauagaag

SEQ ID NO: 113 - RNA, 13 nt, Artificial Sequence
  SEQ ID NO 113
  misc_feature (1)..(13): U can be replaced by T. Any base can be replaced with a modified base.
ggcuggaauagaa

SEQ ID NO: 114 - RNA, 13 nt, Artificial Sequence
  SEQ ID NO 114
  misc_feature (1)..(13): U can be replaced by T. Any base can be replaced with a modified base.
gggcuggaauaga

SEQ ID NO: 115 - RNA, 13 nt, Artificial Sequence
  SEQ ID NO 115
  misc_feature (1)..(13): U can be replaced by T. Any base can be replaced with a modified base.
agggcuggaauag

SEQ ID NO: 116 - RNA, 13 nt, Artificial Sequence
  SEQ ID NO 116
  misc_feature (1)..(13): U can be replaced by T. Any base can be replaced with a modified base.
uagggcuggaaua

SEQ ID NO: 117 - RNA, 13 nt, Artificial Sequence
  SEQ ID NO 117
  misc_feature (1)..(13): U can be replaced by T. Any base can be replaced with a modified base.
uuagggcuggaau

SEQ ID NO: 118 - RNA, 13 nt, Artificial Sequence
  SEQ ID NO 118
  misc_feature (1)..(13): U can be replaced by T. Any base can be replaced with a modified base.
guuagggcuggaa

SEQ ID NO: 119 - RNA, 13 nt, Artificial Sequence
  SEQ ID NO 119
  misc_feature (1)..(13): U can be replaced by T. Any base can be replaced with a modified base.
gguuagggcugga

SEQ ID NO: 120 - RNA, 13 nt, Artificial Sequence
  SEQ ID 120
  misc_feature (1)..(13): U can be replaced by T. Any base can be replaced with a modified base.
ugguuagggcugg

SEQ ID NO: 121 - RNA, 13 nt, Artificial Sequence
  SEQ ID NO 121
  misc_feature (1)..(13): U can be replaced by T. Any base can be replaced with a modified base.
gugguuagggcug

SEQ ID NO: 122 - RNA, 13 nt, Artificial Sequence
  SEQ ID NO 122
  misc_feature (1)..(13): U can be replaced by T. Any base can be replaced with a modified base.
agugguuagggcu

SEQ ID NO: 123 - RNA, 13 nt, Artificial Sequence
  SEQ ID NO 123
  misc_feature (1)..(13): U can be replaced by T. Any base can be replaced with a modified base.
gagugguuagggc

SEQ ID NO: 124 - RNA, 13 nt, Artificial Sequence
  SEQ ID NO 124
  misc_feature (1)..(13): U can be replaced by T. Any base can be replaced with a modified base.
ugagugguuaggg

SEQ ID NO: 125 - RNA, 13 nt, Artificial Sequence
  SEQ ID NO 125
  misc_feature (1)..(13): U can be replaced by T. Any base can be replaced with a modified base.
cugagugguuagg

SEQ ID NO: 126 - RNA, 13 nt, Artificial Sequence
  SEQ ID NO 126
  misc_feature (1)..(13): U can be replaced by T. Any base can be replaced with a modified base.
ccugagugguuag

SEQ ID NO: 127 - RNA, 13 nt, Artificial Sequence
  SEQ ID NO 127
  misc_feature (1)..(13): U can be replaced by T. Any base can be replaced with a modified base.
uccugagugguua

SEQ ID NO: 128 - RNA, 13 nt, Artificial Sequence
  SEQ ID NO 128
  misc_feature (1)..(13): U can be replaced by T. Any base can be replaced with a modified base.
auccugagugguu

SEQ ID NO: 129 - RNA, 13 nt, Artificial Sequence
  SEQ ID NO 129
  misc_feature (1)..(13): U can be replaced by T. Any base can be replaced with a modified base.
aauccugaguggu

SEQ ID NO: 130 - RNA, 13 nt, Artificial Sequence
  SEQ ID NO 130
  misc_feature (1)..(13): U can be replaced by T. Any base can be replaced with a modified base.
caauccugagugg

SEQ ID NO: 131 - RNA, 13 nt, Artificial Sequence
  SEQ ID NO 131
  misc_feature (1)..(13): U can be replaced by T. Any base can be replaced with a modified base.
ccaauccugagug

SEQ ID NO: 132 - RNA, 13 nt, Artificial Sequence
  SEQ ID NO 132
  misc_feature (1)..(13): U can be replaced by T. Any base can be replaced with a modified base.
cccaauccugagu

SEQ ID NO: 133 - RNA, 13 nt, Artificial Sequence
  SEQ ID NO 133
  misc_feature (1)..(13): U can be replaced by T. Any base can be replaced with a modified base.
gcccaauccugag

SEQ ID NO: 134 - RNA, 13 nt, Artificial Sequence
  SEQ ID NO 135
  misc_feature (1)..(13): U can be replaced by T. Any base can be replaced with a modified base.
ggcccaauccuga

SEQ ID NO: 135 - RNA, 13 nt, Artificial Sequence
  SEQ ID NO 135
  misc_feature (1)..(13): U can be replaced by T. Any base can be replaced with a modified base.
cggcccaauccug

SEQ ID NO: 136 - RNA, 13 nt, Artificial Sequence
  SEQ ID NO 136
  misc_feature (1)..(13): U can be replaced by T. Any base can be replaced with a modified base.
acggcccaauccu

SEQ ID NO: 137 - RNA, 13 nt, Artificial Sequence
  SEQ ID NO 137
  misc_feature (1)..(13): U can be replaced by T. Any base can be replaced with a modified base.
aacggcccaaucc

SEQ ID NO: 138 - RNA, 13 nt, Artificial Sequence
  SEQ ID NO 138
  misc_feature (1)..(13): U can be replaced by T. Any base can be replaced with a modified base.
aaacggcccaauc

SEQ ID NO: 139 - RNA, 13 nt, Artificial Sequence
  SEQ ID NO 139
  misc_feature (1)..(13): U can be replaced by T. Any base can be replaced with a modified base.
caaacggcccaau

SEQ ID NO: 140 - RNA, 13 nt, Artificial Sequence
  SEQ ID NO 140
  misc_feature (1)..(13): U can be replaced by T. Any base can be replaced with a modified base.
acaaacggcccaa

SEQ ID NO: 141 - RNA, 13 nt, Artificial Sequence
  SEQ ID NO 141
  misc_feature (1)..(13): U can be replaced by T. Any base can be replaced with a modified base.
cacaaacggccca

SEQ ID NO: 142 - RNA, 13 nt, Artificial Sequence
  SEQ ID NO 142
  misc_feature (1)..(13): U can be replaced by T. Any base can be replaced with a modified base.
acacaaacggccc

SEQ ID NO: 143 - RNA, 13 nt, Artificial Sequence
  SEQ ID NO 143
  misc_feature (1)..(13): U can be replaced by T. Any base can be replaced with a modified base.
gacacaaacggcc

SEQ ID NO: 144 - RNA, 13 nt, Artificial Sequence
  SEQ ID NO 144
  misc_feature (1)..(13): U can be replaced by T. Any base can be replaced with a modified base.
agacacaaacggc

SEQ ID NO: 145 - RNA, 13 nt, Artificial Sequence
  SEQ IF NO 145
  misc_feature (1)..(13): U can be replaced by T. Any base can be replaced with a modified base.
cagacacaaacgg

SEQ ID NO: 146 - RNA, 13 nt, Artificial Sequence
  SEQ ID NO 146
  misc_feature (1)..(13): U can be replaced by T. Any base can be replaced with a modified base.
ccagacacaaacg

SEQ ID NO: 147 - RNA, 13 nt, Artificial Sequence
  SEQ ID NO 147
  misc_feature (1)..(13): U can be replaced by T. Any base can be replaced with a modified base.
cccagacacaaac

SEQ ID NO: 148 - RNA, 13 nt, Artificial Sequence
  SEQ ID NO 148
  misc_feature (1)..(13): U can be replaced by T. Any base can be replaced with a modified base.
acccagacacaaa

SEQ ID NO: 149 - RNA, 13 nt, Artificial Sequence
  SEQ ID NO 149
  misc_feature (1)..(13): U can be replaced by T. Any base can be replaced with a modified base.
uacccagacacaa

SEQ ID NO: 150 - RNA, 13 nt, Artificial Sequence
  SEQ ID NO 150
  misc_feature (1)..(13): U can be replaced by T. Any base can be replaced with a modified base.
auacccagacaca

SEQ ID NO: 151 - RNA, 13 nt, Artificial Sequence
  SEQ ID NO 151
  misc_feature (1)..(13): U can be replaced by T. Any base can be replaced with a modified base.
cauacccagacac

SEQ ID NO: 152 - RNA, 13 nt, Artificial Sequence
  SEQ ID NO 152
  misc_feature (1)..(13): U can be replaced by T. Any base can be replaced with a modified base.
acauacccagaca

SEQ ID NO: 153 - RNA, 13 nt, Artificial Sequence
  SEQ ID NO 153
  misc_feature (1)..(13): U can be replaced by T. Any base can be replaced with a modified base.
gacauacccagac

SEQ ID NO: 154 - RNA, 13 nt, Artificial Sequence
  SEQ ID NO 154
  misc_feature (1)..(13): U can be replaced by T. Any base can be replaced with a modified base.
agacauacccaga

SEQ ID NO: 155 - RNA, 13 nt, Artificial Sequence
  SEQ ID NO 155
  misc_feature (1)..(13): U can be replaced by T. Any base can be replaced with a modified base.
gagacauacccag

SEQ ID NO: 156 - RNA, 13 nt, Artificial Sequence
  SEQ ID NO 156
  misc_feature (1)..(13): U can be replaced by T. Any base can be replaced with a modified base.
agagacauaccca

SEQ ID NO: 157 - RNA, 13 nt, Artificial Sequence
  SEQ ID NO 157
  misc_feature (1)..(13): U can be replaced by T. Any base can be replaced with a modified base.
aagagacauaccc

SEQ ID NO: 158 - RNA, 13 nt, Artificial Sequence
  SEQ ID NO 158
  misc_feature (1)..(13): U can be replaced by T. Any base can be replaced with a modified base.
gaagagacauacc

SEQ ID NO: 159 - RNA, 13 nt, Artificial Sequence
  SEQ ID NO 159
  misc_feature (1)..(13): U can be replaced by T. Any base can be replaced with a modified base.
ggaagagacauac

SEQ ID NO: 160 - RNA, 13 nt, Artificial Sequence
  SEQ ID NO 160
  misc_feature (1)..(13): U can be replaced by T. Any base can be replaced with a modified base.
uggaagagacaua

SEQ ID NO: 161 - RNA, 13 nt, Artificial Sequence
  SEQ ID NO 161
  misc_feature (1)..(13): U can be replaced by T. Any base can be replaced with a modified base.
cuggaagagacau

SEQ ID NO: 162 - RNA, 13 nt, Artificial Sequence
  SEQ ID NO 161
  misc_feature (1)..(13): U can be replaced by T. Any base can be replaced with a modified base.
gcuggaagagaca

SEQ ID NO: 163 - RNA, 13 nt, Artificial Sequence
  SEQ ID NO 163
  misc_feature (1)..(13): U can be replaced by T. Any base can be replaced with a modified base.
agcuggaagagac

SEQ ID NO: 164 - RNA, 13 nt, Artificial Sequence
  SEQ ID NO 164
cagcuggaagaga

SEQ ID NO: 165 - RNA, 13 nt, Artificial Sequence
  SEQ ID NO 165
  misc_feature (1)..(13): U can be replaced by T. Any base can be replaced with a modified base.
gcagcuggaagag

SEQ ID NO: 166 - RNA, 13 nt, Artificial Sequence
  SEQ ID NO 166
  misc_feature (1)..(13): U can be replaced by T. Any base can be replaced with a modified base.
ggcagcuggaaga

SEQ ID NO: 167 - RNA, 13 nt, Artificial Sequence
  SEQ ID NO 167
  misc_feature (1)..(13): U can be replaced by T. Any base can be replaced with a modified base.
aggcagcuggaag

SEQ ID NO: 168 - RNA, 13 nt, Artificial Sequence
  SEQ ID NO 169
  misc_feature (1)..(13): U can be replaced by T. Any base can be replaced with a modified base.
caggcagcuggaa

SEQ ID NO: 169 - RNA, 13 nt, Artificial Sequence
  SEQ ID NO 169
  misc_feature (1)..(13): U can be replaced by T. Any base can be replaced with a modified base.
ccaggcagcugga

SEQ ID NO: 170 - RNA, 13 nt, Artificial Sequence
  SEQ ID NO 170
  misc_feature (1)..(13): U can be replaced by T. Any base can be replaced with a modified base.
cccaggcagcugg

SEQ ID NO: 171 - RNA, 13 nt, Artificial Sequence
  SEQ ID NO 171
  misc_feature (1)..(13): U can be replaced by T. Any base can be replaced with a modified base.
acccaggcagcug

SEQ ID NO: 172 - RNA, 13 nt, Artificial Sequence
  SEQ ID NO 172
  misc_feature (1)..(13): U can be replaced by T. Any base can be replaced with a modified base.
aacccaggcagcu

SEQ ID NO: 173 - RNA, 13 nt, Artificial Sequence
  SEQ ID NO 173
  misc_feature (1)..(13): U can be replaced by T. Any base can be replaced with a modified base.
aaacccaggcagc

SEQ ID NO: 174 - RNA, 13 nt, Artificial Sequence
  SEQ ID NO 174
  misc_feature (1)..(13): U can be replaced by T. Any base can be replaced with a modified base.
gaaacccaggcag

SEQ ID NO: 175 - RNA, 13 nt, Artificial Sequence
  SEQ ID NO 175
  misc_feature (1)..(13): U can be replaced by T. Any base can be replaced with a modified base.
ggaaacccaggca

SEQ ID NO: 176 - RNA, 13 nt, Artificial Sequence
  SEQ ID NO 176
  misc_feature (1)..(13): U can be replaced by T. Any base can be replaced with a modified base.
aggaaacccaggc

SEQ ID NO: 177 - RNA, 13 nt, Artificial Sequence
  SEQ ID NO 177
  misc_feature (1)..(13): U can be replaced by T. Any base can be replaced with a modified base.
caggaaacccagg

SEQ ID NO: 178 - RNA, 13 nt, Artificial Sequence
  SEQ IS NO 178
  misc_feature (1)..(13): U can be replaced by T. Any base can be replaced with a modified base.
ccaggaaacccag

SEQ ID NO: 179 - RNA, 13 nt, Artificial Sequence
  SEQ ID NO 179
  misc_feature (1)..(13): U can be replaced by T. Any base can be replaced with a modified base.
uccaggaaaccca

SEQ ID NO: 180 - RNA, 13 nt, Artificial Sequence
  SEQ ID NO 180
  misc_feature (1)..(13): U can be replaced by T. Any base can be replaced with a modified base.
uuccaggaaaccc

SEQ ID NO: 181 - RNA, 13 nt, Artificial Sequence
  SEQ ID NO 181
  misc_feature (1)..(13): U can be replaced by T. Any base can be replaced with a modified base.
uuuccaggaaacc

SEQ ID NO: 182 - RNA, 13 nt, Artificial Sequence
  SEQ ID NO 182
  misc_feature (1)..(13): U can be replaced by T. Any base can be replaced with a modified base.
cuuuccaggaaac

SEQ ID NO: 183 - RNA, 13 nt, Artificial Sequence
  SEQ ID NO 183
  misc_feature (1)..(13): U can be replaced by T. Any base can be replaced with a modified base.
ucuuuccaggaaa

SEQ ID NO: 184 - RNA, 13 nt, Artificial Sequence
  SEQ ID NO 184
  misc_feature (1)..(13): U can be replaced by T. Any base can be replaced with a modified base.
uucuuuccaggaa

SEQ ID NO: 185 - RNA, 13 nt, Artificial Sequence
  SEQ ID NO 185
  misc_feature (1)..(13): U can be replaced by T. Any base can be replaced with a modified base.
guucuuuccagga

SEQ ID NO: 186 - RNA, 13 nt, Artificial Sequence
  SEQ ID NO 186
  misc_feature (1)..(13): U can be replaced by T. Any base can be replaced with a modified base.
aguucuuuccagg

SEQ ID NO: 187 - RNA, 13 nt, Artificial Sequence
  SEQ ID NO 187
  misc_feature (1)..(13): U can be replaced by T. Any base can be replaced with a modified base.
gaguucuuuccag

SEQ ID NO: 188 - RNA, 13 nt, Artificial Sequence
  SEQ ID NO 188
  misc_feature (1)..(13): U can be replaced by T. Any base can be replaced with a modified base.
agaguucuuucca

SEQ ID NO: 189 - RNA, 13 nt, Artificial Sequence
  SEQ ID NO 189
  misc_feature (1)..(13): U can be replaced by T. Any base can be replaced with a modified base.
aagaguucuuucc

SEQ ID NO: 190 - RNA, 13 nt, Artificial Sequence
  SEQ ID NO 190
  misc_feature (1)..(13): U can be replaced by T. Any base can be replaced with a modified base.
uaagaguucuuuc

SEQ ID NO: 191 - RNA, 13 nt, Artificial Sequence
  SEQ ID NO 191
  misc_feature (1)..(13): U can be replaced by T. Any base can be replaced with a modified base.
auaagaguucuuu

SEQ ID NO: 192 - RNA, 13 nt, Artificial Sequence
  SEQ ID NO 192
  misc_feature (1)..(13): U can be replaced by T. Any base can be replaced with a modified base.
gauaagaguucuu

SEQ ID NO: 193 - RNA, 13 nt, Artificial Sequence
  SEQ ID NO 193
  misc_feature (1)..(13): U can be replaced by T. Any base can be replaced with a modified base.
ggauaagaguucu

SEQ ID NO: 194 - RNA, 13 nt, Artificial Sequence
  SEQ ID NO 194
  misc_feature (1)..(13): U can be replaced by T. Any base can be replaced with a modified base.
gggauaagaguuc

SEQ ID NO: 195 - RNA, 13 nt, Artificial Sequence
  SEQ ID NO 195
  misc_feature (1)..(13): U can be replaced by T. Any base can be replaced with a modified base.
ggggauaagaguu

SEQ ID NO: 196 - RNA, 13 nt, Artificial Sequence
  SEQ ID NO 196
  misc_feature (1)..(13): U can be replaced by T. Any base can be replaced with a modified base.
uggggauaagagu

SEQ ID NO: 197 - RNA, 13 nt, Artificial Sequence
  SEQ ID NO 197
  misc_feature (1)..(13): U can be replaced by T. Any base can be replaced with a modified base.
cuggggauaagag

SEQ ID NO: 198 - RNA, 13 nt, Artificial Sequence
  SEQ ID NO 198
  misc_feature (1)..(13): U can be replaced by T. Any base can be replaced with a modified base.
ccuggggauaaga

SEQ ID NO: 199 - RNA, 13 nt, Artificial Sequence
  SEQ ID NO 199
  misc_feature (1)..(13): U can be replaced by T. Any base can be replaced with a modified base.
uccuggggauaag

SEQ ID NO: 200 - RNA, 13 nt, Artificial Sequence
  SEQ ID NO 200
  misc_feature (1)..(13): U can be replaced by T. Any base can be replaced with a modified base.
uuccuggggauaa

SEQ ID NO: 201 - RNA, 13 nt, Artificial Sequence
  SEQ ID NO 201
  misc_feature (1)..(13): U can be replaced by T. Any base can be replaced with a modified base.
guuccuggggaua

SEQ ID NO: 202 - RNA, 13 nt, Artificial Sequence
  SEQ ID NO 202
  misc_feature (1)..(13): U can be replaced by T. Any base can be replaced with a modified base.
aguuccuggggau

SEQ ID NO: 203 - RNA, 13 nt, Artificial Sequence
  SEQ ID NO 203
  misc_feature (1)..(13): U can be replaced by T. Any base can be replaced with a modified base.
uaguuccugggga

SEQ ID NO: 204 - RNA, 13 nt, Artificial Sequence
  SEQ ID NO 204
  misc_feature (1)..(13): U can be replaced by T. Any base can be replaced with a modified base.
cuaguuccugggg

SEQ ID NO: 205 - RNA, 13 nt, Artificial Sequence
  SEQ ID NO 205
  misc_feature (1)..(13): U can be replaced by T. Any base can be replaced with a modified base.
acuaguuccuggg

SEQ ID NO: 206 - RNA, 13 nt, Artificial Sequence
  SEQ ID NO 207
  misc_feature (1)..(13): U can be replaced by T. Any base can be replaced with a modified base.
aacuaguuccugg

SEQ ID NO: 207 - RNA, 13 nt, Artificial Sequence
  SEQ ID NO 207
  misc_feature (1)..(13): U can be replaced by T. Any base can be replaced with a modified base.
aaacuaguuccug

SEQ ID NO: 208 - RNA, 13 nt, Artificial Sequence
  SEQ ID NO 208
  misc_feature (1)..(13): U can be replaced by T. Any base can be replaced with a modified base.
caaacuaguuccu

SEQ ID NO: 209 - RNA, 13 nt, Artificial Sequence
  SEQ ID NO 209
  misc_feature (1)..(13): U can be replaced by T. Any base can be replaced with a modified base.
acaaacuaguucc

SEQ ID NO: 210 - RNA, 13 nt, Artificial Sequence
  SEQ ID NO 210
  misc_feature (1)..(13): U can be replaced by T. Any base can be replaced with a modified base.
aacaaacuaguuc

SEQ ID NO: 211 - RNA, 13 nt, Artificial Sequence
  SEQ ID NO 211
  misc_feature (1)..(13): U can be replaced by T. Any base can be replaced with a modified base.
caacaaacuaguu

SEQ ID NO: 212 - RNA, 13 nt, Artificial Sequence
  SEQ ID NO 212
  misc_feature (1)..(13): U can be replaced by T. Any base can be replaced with a modified base.
ucaacaaacuagu

SEQ ID NO: 213 - RNA, 13 nt, Artificial Sequence
  SEQ ID NO 213
  misc_feature (1)..(13): U can be replaced by T. Any base can be replaced with a modified base.
uucaacaaacuag

SEQ ID NO: 214 - RNA, 13 nt, Artificial Sequence
  SEQ ID NO 214
  misc_feature (1)..(13): U can be replaced by T. Any base can be replaced with a modified base.
auucaacaaacua

SEQ ID NO: 215 - RNA, 13 nt, Artificial Sequence
  SEQ ID NO 215
  misc_feature (1)..(13): U can be replaced by T. Any base can be replaced with a modified base.
uauucaacaaacu

SEQ ID NO: 216 - RNA, 13 nt, Artificial Sequence
  SEQ ID NO 216
  misc_feature (1)..(13): U can be replaced by T. Any base can be replaced with a modified base.
uuauucaacaaac

SEQ ID NO: 217 - RNA, 13 nt, Artificial Sequence
  SEQ ID NO 217
  misc_feature (1)..(13): U can be replaced by T. Any base can be replaced with a modified base.
uuuauucaacaaa

SEQ ID NO: 218 - RNA, 13 nt, Artificial Sequence
  SEQ ID NO 218
  misc_feature (1)..(13): U can be replaced by T. Any base can be replaced with a modified base.
auuuauucaacaa

SEQ ID NO: 219 - RNA, 13 nt, Artificial Sequence
  SEQ ID NO 219
  misc_feature (1)..(13): U can be replaced by T. Any base can be replaced with a modified base.
cauuuauucaaca

SEQ ID NO: 220 - RNA, 13 nt, Artificial Sequence
  SEQ ID NO 220
  misc_feature (1)..(13): U can be replaced by T. Any base can be replaced with a modified base.
gcauuuauucaac

SEQ ID NO: 221 - RNA, 13 nt, Artificial Sequence
  SEQ ID NO 221
  misc_feature (1)..(13): U can be replaced by T. Any base can be replaced with a modified base.
agcauuuauucaa

SEQ ID NO: 222 - RNA, 13 nt, Artificial Sequence
  SEQ ID NO 222
  misc_feature (1)..(13): U can be replaced by T. Any base can be replaced with a modified base.
cagcauuuauuca

SEQ ID NO: 223 - RNA, 13 nt, Artificial Sequence
  SEQ ID NO 223
  misc_feature (1)..(13): U can be replaced by T. Any base can be replaced with a modified base.
ccagcauuuauuc

SEQ ID NO: 224 - RNA, 13 nt, Artificial Sequence
  SEQ ID NO 224
  misc_feature (1)..(13): U can be replaced by T. Any base can be replaced with a modified base.
accagcauuuauu

SEQ ID NO: 225 - RNA, 13 nt, Artificial Sequence
  CACCAGCAUUUAU
  misc_feature (1)..(13): U can be replaced by T. Any base can be replaced with a modified base.
caccagcauuuau

SEQ ID NO: 226 - RNA, 13 nt, Artificial Sequence
  SEQ ID NO 226
  misc_feature (1)..(13): U can be replaced by T. Any base can be replaced with a modified base.
ucaccagcauuua

SEQ ID NO: 227 - RNA, 13 nt, Artificial Sequence
  SEQ ID NO 227
  misc_feature (1)..(13): U can be replaced by T. Any base can be replaced with a modified base.
uucaccagcauuu

SEQ ID NO: 228 - RNA, 13 nt, Artificial Sequence
  SEQ ID NO 228
  misc_feature (1)..(13): U can be replaced by T. Any base can be replaced with a modified base.
auucaccagcauu

SEQ ID NO: 229 - RNA, 13 nt, Artificial Sequence
  SEQ ID NO 229
  misc_feature (1)..(13): U can be replaced by T. Any base can be replaced with a modified base.
cauucaccagcau

SEQ ID NO: 230 - RNA, 13 nt, Artificial Sequence
  SEQ ID NO 230
  misc_feature (1)..(13): U can be replaced by T. Any base can be replaced with a modified base.
ucauucaccagca

SEQ ID NO: 231 - RNA, 13 nt, Artificial Sequence
  SEQ ID NO 231
  misc_feature (1)..(13): U can be replaced by T. Any base can be replaced with a modified base.
uucauucaccagc

SEQ ID NO: 232 - RNA, 13 nt, Artificial Sequence
  SEQ ID NO 232
  misc_feature (1)..(13): U can be replaced by T. Any base can be replaced with a modified base.
auucauucaccag

SEQ ID NO: 233 - RNA, 13 nt, Artificial Sequence
  SEQ ID NO 233
  misc_feature (1)..(13): U can be replaced by T. Any base can be replaced with a modified base.
cauucauucacca

SEQ ID NO: 234 - RNA, 13 nt, Artificial Sequence
  SEQ ID NO 234
  misc_feature (1)..(13): U can be replaced by T. Any base can be replaced with a modified base.
ucauucauucacc

SEQ ID NO: 235 - RNA, 13 nt, Artificial Sequence
  SEQ ID NO 235
  misc_feature (1)..(13): U can be replaced by T. Any base can be replaced with a modified base.
uucauucauucac

SEQ ID NO: 236 - RNA, 13 nt, Artificial Sequence
  SEQ ID NO 236
  misc_feature (1)..(13): U can be replaced by T. Any base can be replaced with a modified base.
auucauucauuca

SEQ ID NO: 237 - RNA, 13 nt, Artificial Sequence
  SEQ ID NO 237
  misc_feature (1)..(13): U can be replaced by T. Any base can be replaced with a modified base.
cauucauucauuc

SEQ ID NO: 238 - RNA, 13 nt, Artificial Sequence
  SEQ ID NO 238
  misc_feature (1)..(13): U can be replaced by T. Any base can be replaced with a modified base.
ucauucauucauu

SEQ ID NO: 239 - RNA, 13 nt, Artificial Sequence
  SEQ ID NO 239
  misc_feature (1)..(13): U can be replaced by T. Any base can be replaced with a modified base.
aucauucauucau

SEQ ID NO: 240 - RNA, 13 nt, Artificial Sequence
  SEQ ID NO 240
  misc_feature (1)..(13): U can be replaced by T. Any base can be replaced with a modified base.
aaucauucauuca

SEQ ID NO: 241 - RNA, 13 nt, Artificial Sequence
  SEQ ID NO 241
  misc_feature (1)..(13): U can be replaced by T. Any base can be replaced with a modified base.
caaucauucauuc

SEQ ID NO: 242 - RNA, 13 nt, Artificial Sequence
  SEQ ID NO 242
  misc_feature (1)..(13): U can be replaced by T. Any base can be replaced with a modified base.
ucaaucauucauu

SEQ ID NO: 243 - RNA, 13 nt, Artificial Sequence
  SEQ ID NO 243
  misc_feature (1)..(13): U can be replaced by T. Any base can be replaced with a modified base.
uucaaucauucau

SEQ ID NO: 244 - RNA, 13 nt, Artificial Sequence
  SEQ ID NO 244
  misc_feature (1)..(13): U can be replaced by T. Any base can be replaced with a modified base.
guucaaucauuca

SEQ ID NO: 245 - RNA, 13 nt, Artificial Sequence
  SEQ ID NO 245
  misc_feature (1)..(13): U can be replaced by T. Any base can be replaced with a modified base.
uguucaaucauuc

SEQ ID NO: 246 - RNA, 13 nt, Artificial Sequence
  SEQ ID NO 246
  misc_feature (1)..(13): U can be replaced by T. Any base can be replaced with a modified base.
cuguucaaucauu

SEQ ID NO: 247 - RNA, 13 nt, Artificial Sequence
  SEQ ID NO 247
  misc_feature (1)..(13): U can be replaced by T. Any base can be replaced with a modified base.
ucuguucaaucau

SEQ ID NO: 248 - RNA, 13 nt, Artificial Sequence
  SEQ ID NO 248
  misc_feature (1)..(13): U can be replaced by T. Any base can be replaced with a modified base.
aucuguucaauca

SEQ ID NO: 249 - RNA, 13 nt, Artificial Sequence
  SEQ ID NO 249
  misc_feature (1)..(13): U can be replaced by T. Any base can be replaced with a modified base.
caucuguucaauc

SEQ ID NO: 250 - RNA, 13 nt, Artificial Sequence
  SEQ ID NO 250
  misc_feature (1)..(13): U can be replaced by T. Any base can be replaced with a modified base.
ucaucuguucaau

SEQ ID NO: 251 - RNA, 13 nt, Artificial Sequence
  SEQ ID NO 251
  misc_feature (1)..(13): U can be replaced by T. Any base can be replaced with a modified base.
uucaucuguucaa

SEQ ID NO: 252 - RNA, 13 nt, Artificial Sequence
  SEQ ID NO 252
  misc_feature (1)..(13): U can be replaced by T. Any base can be replaced with a modified base.
auucaucuguuca

SEQ ID NO: 253 - RNA, 13 nt, Artificial Sequence
  SEQ ID NO 253
  misc_feature (1)..(13): U can be replaced by T. Any base can be replaced with a modified base.
cauucaucuguuc

SEQ ID NO: 254 - RNA, 13 nt, Artificial Sequence
  SEQ ID NO 254
  misc_feature (1)..(13): U can be replaced by T. Any base can be replaced with a modified base.
ucauucaucuguu

SEQ ID NO: 255 - RNA, 13 nt, Artificial Sequence
  SEQ ID NO 255
  misc_feature (1)..(13): U can be replaced by T. Any base can be replaced with a modified base.
cucauucaucugu

SEQ ID NO: 256 - RNA, 13 nt, Artificial Sequence
  SEQ ID NO 256
  misc_feature (1)..(13): U can be replaced by T. Any base can be replaced with a modified base.
acucauucaucug

SEQ ID NO: 257 - RNA, 13 nt, Artificial Sequence
  SEQ ID NO 257
  misc_feature (1)..(13): U can be replaced by T. Any base can be replaced with a modified base.
cacucauucaucu

SEQ ID NO: 258 - RNA, 13 nt, Artificial Sequence
  SEQ ID NO 258
  misc_feature (1)..(13): U can be replaced by T. Any base can be replaced with a modified base.
ucacucauucauc

SEQ ID NO: 259 - RNA, 13 nt, Artificial Sequence
  SEQ ID NO 259
  misc_feature (1)..(13): U can be replaced by T. Any base can be replaced with a modified base.
aucacucauucau

SEQ ID NO: 260 - RNA, 13 nt, Artificial Sequence
  SEQ ID NO 260
  misc_feature (1)..(13): U can be replaced by T. Any base can be replaced with a modified base.
caucacucauuca

SEQ ID NO: 261 - RNA, 13 nt, Artificial Sequence
  SEQ ID NO 261
  misc_feature (1)..(13): U can be replaced by T. Any base can be replaced with a modified base.
ucaucacucauuc

SEQ ID NO: 262 - RNA, 13 nt, Artificial Sequence
  SEQ ID NO 262
  misc_feature (1)..(13): U can be replaced by T. Any base can be replaced with a modified base.
cucaucacucauu

SEQ ID NO: 263 - RNA, 13 nt, Artificial Sequence
  SEQ ID NO 263
  misc_feature (1)..(13): U can be replaced by T. Any base can be replaced with a modified base.
acucaucacucau

SEQ ID NO: 264 - RNA, 13 nt, Artificial Sequence
  SEQ ID NO 264
  misc_feature (1)..(13): U can be replaced by T. Any base can be replaced with a modified base.
uacucaucacuca

SEQ ID NO: 265 - RNA, 13 nt, Artificial Sequence
  SEQ ID NO 265
  misc_feature (1)..(13): U can be replaced by T. Any base can be replaced with a modified base.
cuacucaucacuc

SEQ ID NO: 266 - RNA, 13 nt, Artificial Sequence
  SEQ ID NO 266
  misc_feature (1)..(13): U can be replaced by T. Any base can be replaced with a modified base.
ucuacucaucacu

SEQ ID NO: 267 - RNA, 13 nt, Artificial Sequence
  SEQ ID NO 267
  misc_feature (1)..(13): U can be replaced by T. Any base can be replaced with a modified base.
aucuacucaucac

SEQ ID NO: 268 - RNA, 13 nt, Artificial Sequence
  SEQ ID NO 268
  misc_feature (1)..(13): U can be replaced by T. Any base can be replaced with a modified base.
uaucuacucauca

SEQ ID NO: 269 - RNA, 13 nt, Artificial Sequence
  SEQ ID NO 260
  misc_feature (1)..(13): U can be replaced by T. Any base can be replaced with a modified base.
uuaucuacucauc

SEQ ID NO: 270 - RNA, 13 nt, Artificial Sequence
  SEQ ID NO 270
  misc_feature (1)..(13): U can be replaced by T. Any base can be replaced with a modified base.
uuuaucuacucau

SEQ ID NO: 271 - RNA, 13 nt, Artificial Sequence
  SEQ ID NO 271
  misc_feature (1)..(13): U can be replaced by T. Any base can be replaced with a modified base.
uuuuaucuacuca

SEQ ID NO: 272 - RNA, 13 nt, Artificial Sequence
  SEQ ID NO 272
  misc_feature (1)..(13): U can be replaced by T. Any base can be replaced with a modified base.
cuuuuaucuacuc

SEQ ID NO: 273 - RNA, 13 nt, Artificial Sequence
  SEQ ID NO 273
  misc_feature (1)..(13): U can be replaced by T. Any base can be replaced with a modified base.
ccuuuuaucuacu

SEQ ID NO: 274 - RNA, 13 nt, Artificial Sequence
  SEQ ID NO 274
  misc_feature (1)..(13): U can be replaced by T. Any base can be replaced with a modified base.
gcuuuuaucuacu

SEQ ID NO: 275 - RNA, 13 nt, Artificial Sequence
  SEQ ID NO 275
  misc_feature (1)..(13): U can be replaced by T. Any base can be replaced with a modified base.
uccuuuuaucuac

SEQ ID NO: 276 - RNA, 13 nt, Artificial Sequence
  SEQ ID NO 276
  misc_feature (1)..(13): U can be replaced by T. Any base can be replaced with a modified base.
ugcuuuuaucuac

SEQ ID NO: 277 - RNA, 13 nt, Artificial Sequence
  SEQ ID NO 277
  misc_feature (1)..(13): U can be replaced by T. Any base can be replaced with a modified base.
auccuuuuaucua

SEQ ID NO: 278 - RNA, 13 nt, Artificial Sequence
  SEQ ID NO 278
  misc_feature (1)..(13): U can be replaced by T. Any base can be replaced with a modified base.
augcuuuuaucua

SEQ ID NO: 279 - RNA, 13 nt, Artificial Sequence
  SEQ ID NO 279
  misc_feature (1)..(13): U can be replaced by T. Any base can be replaced with a modified base.
cauccuuuuaucu

SEQ ID NO: 280 - RNA, 13 nt, Artificial Sequence
  SEQ ID NO 280
  misc_feature (1)..(13): U can be replaced by T. Any base can be replaced with a modified base.
caugcuuuuaucu

SEQ ID NO: 281 - RNA, 13 nt, Artificial Sequence
  SEQ ID NO 281
ccauccuuuuauc

SEQ ID NO: 282 - RNA, 13 nt, Artificial Sequence
  SEQ ID NO 282
  misc_feature (1)..(13): U can be replaced by T. Any base can be replaced with a modified base.
ccaugcuuuuauc

SEQ ID NO: 283 - RNA, 13 nt, Artificial Sequence
  SEQ ID NO 283
  misc_feature (1)..(13): U can be replaced by T. Any base can be replaced with a modified base.
uccauccuuuuau

SEQ ID NO: 284 - RNA, 13 nt, Artificial Sequence
  SEQ ID NO 284
  misc_feature (1)..(13): U can be replaced by T. Any base can be replaced with a modified base.
uccaugcuuuuau

SEQ ID NO: 285 - RNA, 13 nt, Artificial Sequence
  SEQ ID NO 285
  misc_feature (1)..(13): U can be replaced by T. Any base can be replaced with a modified base.
auccauccuuuua

SEQ ID NO: 286 - RNA, 13 nt, Artificial Sequence
  SEQ ID NO 286
  misc_feature (1)..(13): U can be replaced by T. Any base can be replaced with a modified base.
auccaugcuuuua

SEQ ID NO: 287 - RNA, 13 nt, Artificial Sequence
  SEQ ID No 287
  misc_feature (1)..(13): U can be replaced by T. Any base can be replaced with a modified base.
cauccauccuuuu

SEQ ID NO: 288 - RNA, 13 nt, Artificial Sequence
  SEQ ID NO 288
  misc_feature (1)..(13): U can be replaced by T. Any base can be replaced with a modified base.
cauccaugcuuuu

SEQ ID NO: 289 - RNA, 13 nt, Artificial Sequence
  SEQ ID NO 289
  misc_feature (1)..(13): U can be replaced by T. Any base can be replaced with a modified base.
ccauccauccuuu

SEQ ID NO: 290 - RNA, 13 nt, Artificial Sequence
  SEQ ID NO 290
  misc_feature (1)..(13): U can be replaced by T. Any base can be replaced with a modified base.
ccauccaugcuuu

SEQ ID NO: 291 - RNA, 13 nt, Artificial Sequence
  SEQ ID NO 291
  misc_feature (1)..(13): U can be replaced by T. Any base can be replaced with a modified base.
uccauccauccuu

SEQ ID NO: 292 - RNA, 13 nt, Artificial Sequence
  SEQ ID NO 292
  misc_feature (1)..(13): U can be replaced by T. Any base can be replaced with a modified base.
uccauccaugcuu

SEQ ID NO: 293 - RNA, 13 nt, Artificial Sequence
  SEQ ID NO 293
  misc_feature (1)..(13): U can be replaced by T. Any base can be replaced with a modified base.
cuccauccauccu

SEQ ID NO: 294 - RNA, 13 nt, Artificial Sequence
  SEQ ID NO 294
  misc_feature (1)..(13): U can be replaced by T. Any base can be replaced with a modified base.
cuccauccaugcu

SEQ ID NO: 295 - RNA, 13 nt, Artificial Sequence
  SEQ ID NO 295
  misc_feature (1)..(13): U can be replaced by T. Any base can be replaced with a modified base.
ucuccauccaucc

SEQ ID NO: 296 - RNA, 13 nt, Artificial Sequence
  SEQ ID NO 296
  misc_feature (1)..(13): U can be replaced by T. Any base can be replaced with a modified base.
ucuccauccaugc

SEQ ID NO: 297 - RNA, 13 nt, Artificial Sequence
  SEQ ID NO 297
  misc_feature (1)..(13): U can be replaced by T. Any base can be replaced with a modified base.
cucuccauccauc

SEQ ID NO: 298 - RNA, 13 nt, Artificial Sequence
  SEQ ID NO 298
  misc_feature (1)..(13): U can be replaced by T. Any base can be replaced with a modified base.
cucuccauccaug

SEQ ID NO: 299 - RNA, 13 nt, Artificial Sequence
  SEQ ID NO 299
  misc_feature (1)..(13): U can be replaced by T. Any base can be replaced with a modified base.
ucucuccauccau

SEQ ID NO: 300 - RNA, 13 nt, Artificial Sequence
  SEQ ID NO 300
  misc_feature (1)..(13): U can be replaced by T. Any base can be replaced with a modified base.
aucucuccaucca

SEQ ID NO: 301 - RNA, 13 nt, Artificial Sequence
  SEQ ID NO 301
  misc_feature (1)..(13): U can be replaced by T. Any base can be replaced with a modified base.
caucucuccaucc

SEQ ID NO: 302 - RNA, 13 nt, Artificial Sequence
  SEQ ID NO 302
  misc_feature (1)..(13): U can be replaced by T. Any base can be replaced with a modified base.
ccaucucuccauc

SEQ ID NO: 303 - RNA, 13 nt, Artificial Sequence
  SEQ ID NO 303
  misc_feature (1)..(13): U can be replaced by T. Any base can be replaced with a modified base.
cccaucucuccau

SEQ ID NO: 304 - RNA, 13 nt, Artificial Sequence
  SEQ ID NO 304
  misc_feature (1)..(13): U can be replaced by T. Any base can be replaced with a modified base.
acccaucucucca

SEQ ID NO: 305 - RNA, 13 nt, Artificial Sequence
  SEQ ID NO 305
  misc_feature (1)..(13): U can be replaced by T. Any base can be replaced with a modified base.
cacccaucucucc

SEQ ID NO: 306 - RNA, 13 nt, Artificial Sequence
  SEQ ID NO 306
  misc_feature (1)..(13): U can be replaced by T. Any base can be replaced with a modified base.
ucacccaucucuc

SEQ ID NO: 307 - RNA, 13 nt, Artificial Sequence
  SEQ ID NO 307
  misc_feature (1)..(13): U can be replaced by T. Any base can be replaced with a modified base.
cucacccaucucu

SEQ ID NO: 308 - RNA, 13 nt, Artificial Sequence
  SEQ ID NO 308
  misc_feature (1)..(13): U can be replaced by T. Any base can be replaced with a modified base.
acucacccaucuc

SEQ ID NO: 309 - RNA, 13 nt, Artificial Sequence
  SEQ ID NO 309
  misc_feature (1)..(13): U can be replaced by T. Any base can be replaced with a modified base.
uacucacccaucu

SEQ ID NO: 310 - RNA, 13 nt, Artificial Sequence
  SEQ ID NO 310
  misc_feature (1)..(13): U can be replaced by T. Any base can be replaced with a modified base.
guacucacccauc

SEQ ID NO: 311 - RNA, 13 nt, Artificial Sequence
  SEQ ID NO 311
  misc_feature (1)..(13): U can be replaced by T. Any base can be replaced with a modified base.
uguacucacccau

SEQ ID NO: 312 - RNA, 13 nt, Artificial Sequence
  SEQ ID NO 312
  misc_feature (1)..(13): U can be replaced by T. Any base can be replaced with a modified base.
auguacucaccca

SEQ ID NO: 313 - RNA, 13 nt, Artificial Sequence
  SEQ ID NO 313
  misc_feature (1)..(13): U can be replaced by T. Any base can be replaced with a modified base.
cauguacucaccc

SEQ ID NO: 314 - RNA, 13 nt, Artificial Sequence
  SEQ ID NO 314
  misc_feature (1)..(13): U can be replaced by T. Any base can be replaced with a modified base.
ccauguacucacc

SEQ ID NO: 315 - RNA, 13 nt, Artificial Sequence
  SEQ ID NO 315
  misc_feature (1)..(13): U can be replaced by T. Any base can be replaced with a modified base.
uccauguacucac

SEQ ID NO: 316 - RNA, 13 nt, Artificial Sequence
  SEQ ID NO 316
  misc_feature (1)..(13): U can be replaced by T. Any base can be replaced with a modified base.
auccauguacuca

SEQ ID NO: 317 - RNA, 13 nt, Artificial Sequence
  SEQ ID NO 317
  misc_feature (1)..(13): U can be replaced by T. Any base can be replaced with a modified base.
cauccauguacuc

SEQ ID NO: 318 - RNA, 13 nt, Artificial Sequence
  SEQ ID NO 318
  misc_feature (1)..(13): U can be replaced by T. Any base can be replaced with a modified base.
ccauccauguacu

SEQ ID NO: 319 - RNA, 13 nt, Artificial Sequence
  SEQ ID NO 319
  misc_feature (1)..(13): U can be replaced by T. Any base can be replaced with a modified base.
uccauccauguac

SEQ ID NO: 320 - RNA, 13 nt, Artificial Sequence
  SEQ ID NO 320
  misc_feature (1)..(13): U can be replaced by T. Any base can be replaced with a modified base.
auccauccaugua

SEQ ID NO: 321 - RNA, 13 nt, Artificial Sequence
  SEQ ID NO 321
  misc_feature (1)..(13): U can be replaced by T. Any base can be replaced with a modified base.
uauccauccaugu

SEQ ID NO: 322 - RNA, 13 nt, Artificial Sequence
  SEQ ID NO 322
  misc_feature (1)..(13): U can be replaced by T. Any base can be replaced with a modified base.
cuauccauccaug

SEQ ID NO: 323 - RNA, 13 nt, Artificial Sequence
  SEQ ID NO 323
  misc_feature (1)..(13): U can be replaced by T. Any base can be replaced with a modified base.
ucuauccauccau

SEQ ID NO: 324 - RNA, 13 nt, Artificial Sequence
  SEQ ID NO 324
  misc_feature (1)..(13): U can be replaced by T. Any base can be replaced with a modified base.
aucuauccaucca

SEQ ID NO: 325 - RNA, 13 nt, Artificial Sequence
  SEQ ID NO 325
  misc_feature (1)..(13): U can be replaced by T. Any base can be replaced with a modified base.
caucuauccaucc

SEQ ID NO: 326 - RNA, 13 nt, Artificial Sequence
  SEQ ID NO 326
  misc_feature (1)..(13): U can be replaced by T. Any base can be replaced with a modified base.
ccaucuauccauc

SEQ ID NO: 327 - RNA, 13 nt, Artificial Sequence
  SEQ ID NO 327
  misc_feature (1)..(13): U can be replaced by T. Any base can be replaced with a modified base.
uccaucuauccau

SEQ ID NO: 328 - RNA, 13 nt, Artificial Sequence
  SEQ ID NO 328
  misc_feature (1)..(13): U can be replaced by T. Any base can be replaced with a modified base.
auccaucuaucca

SEQ ID NO: 329 - RNA, 13 nt, Artificial Sequence
  SEQ ID NO 329
  misc_feature (1)..(13): U can be replaced by T. Any base can be replaced with a modified base.
cauccaucuaucc

SEQ ID NO: 330 - RNA, 13 nt, Artificial Sequence
  SEQ ID NO 330
  misc_feature (1 )..(13): U can be replaced by T. Any base can be replaced with a modified base.
ucauccaucuauc

SEQ ID NO: 331 - RNA, 13 nt, Artificial Sequence
  SEQ ID NO 331
  misc_feature (1)..(13): U can be replaced by T. Any base can be replaced with a modified base.
cucauccaucuau

SEQ ID NO: 332 - RNA, 13 nt, Artificial Sequence
  SEQ ID NO 332
  misc_feature (1)..(13): U can be replaced by T. Any base can be replaced with a modified base.
acucauccaucua

SEQ ID NO: 333 - RNA, 13 nt, Artificial Sequence
  SEQ ID NO 333
  misc_feature (1)..(13): U can be replaced by T. Any base can be replaced with a modified base.
aacucauccaucu

SEQ ID NO: 334 - RNA, 13 nt, Artificial Sequence
  SEQ ID NO 334
  misc_feature (1)..(13): U can be replaced by T. Any base can be replaced with a modified base.
caacucauccauc

SEQ ID NO: 335 - RNA, 13 nt, Artificial Sequence
  SEQ ID NO 335
  misc_feature (1)..(13): U can be replaced by T. Any base can be replaced with a modified base.
ccaacucauccau

SEQ ID NO: 336 - RNA, 13 nt, Artificial Sequence
  SEQ ID NO 336
  misc_feature (1)..(13): U can be replaced by T. Any base can be replaced with a modified base.
accaacucaucca

SEQ ID NO: 337 - RNA, 13 nt, Artificial Sequence
  SEQ ID NO 337
  misc_feature (1)..(13): U can be replaced by T. Any base can be replaced with a modified base.
caccaacucaucc

SEQ ID NO: 338 - RNA, 13 nt, Artificial Sequence
  SEQ ID NO 338
  misc_feature (1)..(13): U can be replaced by T. Any base can be replaced with a modified base.
ccaccaacucauc

SEQ ID NO: 339 - RNA, 13 nt, Artificial Sequence
  SEQ ID NO 339
  misc_feature (1)..(13): U can be replaced by T. Any base can be replaced with a modified base.
cccaccaacucau

SEQ ID NO: 340 - RNA, 13 nt, Artificial Sequence
  SEQ ID NO 340
  misc_feature (1)..(13): U can be replaced by T. Any base can be replaced with a modified base.
acccaccaacuca

SEQ ID NO: 341 - RNA, 13 nt, Artificial Sequence
  SEQ ID NO 341
  misc_feature (1)..(13): U can be replaced by T. Any base can be replaced with a modified base.
uacccaccaacuc

SEQ ID NO: 342 - RNA, 13 nt, Artificial Sequence
  SEQ ID NO 342
  misc_feature (1)..(13): U can be replaced by T. Any base can be replaced with a modified base.
cuacccaccaacu

SEQ ID NO: 343 - RNA, 13 nt, Artificial Sequence
  SEQ ID NO 343
  misc_feature (1)..(13): U can be replaced by T. Any base can be replaced with a modified base.
ucuacccaccaac

SEQ ID NO: 344 - RNA, 13 nt, Artificial Sequence
  SEQ ID NO 344
  misc_feature (1)..(13): U can be replaced by T. Any base can be replaced with a modified base.
aucuacccaccaa

SEQ ID NO: 345 - RNA, 13 nt, Artificial Sequence
  SEQ ID NO 345
  misc_feature (1)..(13): U can be replaced by T. Any base can be replaced with a modified base.
aaucuacccacca

SEQ ID NO: 346 - RNA, 13 nt, Artificial Sequence
  SEQ ID NO 346
  misc_feature (1)..(13): U can be replaced by T. Any base can be replaced with a modified base.
gaaucuacccacc

SEQ ID NO: 347 - RNA, 13 nt, Artificial Sequence
  SEQ ID NO 347
cgaaucuacccac

SEQ ID NO: 348 - RNA, 13 nt, Artificial Sequence
  SEQ ID NO 348
acgaaucuaccca

SEQ ID NO: 349 - RNA, 13 nt, Artificial Sequence
  SEQ ID NO 349
  misc_feature (1)..(13): U can be replaced by T. Any base can be replaced with a modified base.
cacgaaucuaccc

SEQ ID NO: 350 - RNA, 13 nt, Artificial Sequence
  SEQ ID NO 350
  misc_feature (1)..(13): U can be replaced by T. Any base can be replaced with a modified base.
ccacgaaucuacc

SEQ ID NO: 351 - RNA, 13 nt, Artificial Sequence
  SEQ ID NO 351
  misc_feature (1)..(13): U can be replaced by T. Any base can be replaced with a modified base.
gccacgaaucuac

SEQ ID NO: 352 - RNA, 13 nt, Artificial Sequence
  SEQ ID NO 352
  misc_feature (1)..(13): U can be replaced by T. Any base can be replaced with a modified base.
agccacgaaucua

SEQ ID NO: 353 - RNA, 13 nt, Artificial Sequence
  SEQ ID NO 353
  misc_feature (1)..(13): U can be replaced by T. Any base can be replaced with a modified base.
cagccacucacaa

SEQ ID NO: 354 - RNA, 13 nt, Artificial Sequence
  SEQ ID NO 354
  misc_feature (1)..(13): U can be replaced by T. Any base can be replaced with a modified base.
ccagccacucaca

SEQ ID NO: 355 - RNA, 13 nt, Artificial Sequence
  SEQ ID NO 355
  misc_feature (1)..(13): U can be replaced by T. Any base can be replaced with a modified base.
accagccacucac

SEQ ID NO: 356 - RNA, 13 nt, Artificial Sequence
  SEQ ID NO 356
  misc_feature (1)..(13): U can be replaced by T. Any base can be replaced with a modified base.
caccagccacuca

SEQ ID NO: 357 - RNA, 13 nt, Artificial Sequence
  SEQ ID NO 357
  misc_feature (1)..(13): U can be replaced by T. Any base can be replaced with a modified base.
ccaccagccacuc

SEQ ID NO: 358 - RNA, 13 nt, Artificial Sequence
  SEQ ID NO 358
  misc_feature (1)..(13): U can be replaced by T. Any base can be replaced with a modified base.
uccaccagccacu

SEQ ID NO: 359 - RNA, 13 nt, Artificial Sequence
  SEQ ID NO 359
  misc_feature (1)..(13): U can be replaced by T. Any base can be replaced with a modified base.
guccaccagccac

SEQ ID NO: 360 - RNA, 13 nt, Artificial Sequence
  SEQ ID NO 360
  misc_feature (1)..(13): U can be replaced by T. Any base can be replaced with a modified base.
uguccaccagcca

SEQ ID NO: 361 - RNA, 13 nt, Artificial Sequence
  SEQ ID NO 361
  misc_feature (1)..(13): U can be replaced by T. Any base can be replaced with a modified base.
cuguccaccagcc

SEQ ID NO: 362 - RNA, 13 nt, Artificial Sequence
  SEQ ID NO 362
  misc_feature (1)..(13): U can be replaced by T. Any base can be replaced with a modified base.
ucuguccaccagc

SEQ ID NO: 363 - RNA, 13 nt, Artificial Sequence
  SEQ ID NO 363
  misc_feature (1)..(13): U can be replaced by T. Any base can be replaced with a modified base.
gucuguccaccag

SEQ ID NO: 364 - RNA, 13 nt, Artificial Sequence
  SEQ ID NO 364
  misc_feature (1)..(13): U can be replaced by T. Any base can be replaced with a modified base.
cgucuguccacca

SEQ ID NO: 365 - RNA, 13 nt, Artificial Sequence
  SEQ ID NO 365
  misc_feature (1)..(13): U can be replaced by T. Any base can be replaced with a modified base.
ucgucuguccacc

SEQ ID NO: 366 - RNA, 13 nt, Artificial Sequence
  SEQ ID No 366
  misc_feature (1)..(13): U can be replaced by T. Any base can be replaced with a modified base.
uucgucuguccac

SEQ ID NO: 367 - RNA, 13 nt, Artificial Sequence
  SEQ ID NO 367
  misc_feature (1)..(13): U can be replaced by T. Any base can be replaced with a modified base.
uuucgucugucca

SEQ ID NO: 368 - RNA, 13 nt, Artificial Sequence
  SEQ ID NO 368
  misc_feature (1)..(13): U can be replaced by T. Any base can be replaced with a modified base.
uuuucgucugucc

SEQ ID NO: 369 - RNA, 13 nt, Artificial Sequence
  SEQ ID NO 369
  misc_feature (1)..(13): U can be replaced by T. Any base can be replaced with a modified base.
uuuuucgucuguc

SEQ ID NO: 370 - RNA, 13 nt, Artificial Sequence
  SEQ ID NO 370
  misc_feature (1)..(13): U can be replaced by T. Any base can be replaced with a modified base.
auuuuucgucugu

SEQ ID NO: 371 - RNA, 13 nt, Artificial Sequence
  SEQ ID NO 371
  misc_feature (1)..(13): U can be replaced by T. Any base can be replaced with a modified base.
cauuuuucgucug

SEQ ID NO: 372 - RNA, 13 nt, Artificial Sequence
  SEQ ID NO 372
  misc_feature (1)..(13): U can be replaced by T. Any base can be replaced with a modified base.
ccauuuuucgucu

SEQ ID NO: 373 - RNA, 13 nt, Artificial Sequence
  SEQ ID NO 373
  misc_feature (1)..(13): U can be replaced by T. Any base can be replaced with a modified base.
uccauuuuucguc

SEQ ID NO: 374 - RNA, 13 nt, Artificial Sequence
  SEQ ID NO 374
  misc_feature (1)..(13): U can be replaced by T. Any base can be replaced with a modified base.
auccauuuuucgu

SEQ ID NO: 375 - RNA, 13 nt, Artificial Sequence
  SEQ ID NO 375
  misc_feature (1)..(13): U can be replaced by T. Any base can be replaced with a modified base.
cauccauuuuucg

SEQ ID NO: 376 - RNA, 13 nt, Artificial Sequence
  SEQ ID NO 376
  misc_feature (1)..(13): U can be replaced by T. Any base can be replaced with a modified base.
ccauccauuuuuc

SEQ ID NO: 377 - RNA, 13 nt, Artificial Sequence
  SEQ ID NO 377
  misc_feature (1)..(13): U can be replaced by T. Any base can be replaced with a modified base.
accauccauuuuu

SEQ ID NO: 378 - RNA, 13 nt, Artificial Sequence
  SEQ ID NO 378
  misc_feature (1)..(13): U can be replaced by T. Any base can be replaced with a modified base.
cccauccauuuuu

SEQ ID NO: 379 - RNA, 13 nt, Artificial Sequence
  SEQ ID NO 379
  misc_feature (1)..(13): U can be replaced by T. Any base can be replaced with a modified base.
aaccauccauuuu

SEQ ID NO: 380 - RNA, 13 nt, Artificial Sequence
  SEQ ID NO 380
  misc_feature (1)..(13): U can be replaced by T. Any base can be replaced with a modified base.
acccauccauuuu

SEQ ID NO: 381 - RNA, 13 nt, Artificial Sequence
  SEQ ID NO 381
  misc_feature (1)..(13): U can be replaced by T. Any base can be replaced with a modified base.
caaccauccauuu

SEQ ID NO: 382 - RNA, 13 nt, Artificial Sequence
  SEQ ID NO 382
  misc_feature (1)..(13): U can be replaced by T. Any base can be replaced with a modified base.
cacccauccauuu

SEQ ID NO: 383 - RNA, 13 nt, Artificial Sequence
  SEQ ID NO 383
  misc_feature (1)..(13): U can be replaced by T. Any base can be replaced with a modified base.
ccaaccauccauu

SEQ ID NO: 384 - RNA, 13 nt, Artificial Sequence
  SEQ ID NO 384
  misc_feature (1)..(13): U can be replaced by T. Any base can be replaced with a modified base.
ccacccauccauu

SEQ ID NO: 385 - RNA, 13 nt, Artificial Sequence
  SEQ ID NO 385
  misc_feature (1)..(13): U can be replaced by T. Any base can be replaced with a modified base.
uccaaccauccau

SEQ ID NO: 386 - RNA, 13 nt, Artificial Sequence
  SEQ ID NO 386
  misc_feature (1)..(13): U can be replaced by T. Any base can be replaced with a modified base.
uccacccauccau

SEQ ID NO: 387 - RNA, 13 nt, Artificial Sequence
  SEQ ID NO 387
  misc_feature (1)..(13): U can be replaced by T. Any base can be replaced with a modified base.
auccaaccaucca

SEQ ID NO: 388 - RNA, 13 nt, Artificial Sequence
  SEQ ID NO 388
  misc_feature (1)..(13): U can be replaced by T. Any base can be replaced with a modified base.
auccacccaucca

SEQ ID NO: 389 - RNA, 13 nt, Artificial Sequence
  SEQ ID NO 389
  misc_feature (1)..(13): U can be replaced by T. Any base can be replaced with a modified base.
uauccaaccaucc

SEQ ID NO: 390 - RNA, 13 nt, Artificial Sequence
  SEQ ID NO 390
  misc_feature (1)..(13): U can be replaced by T. Any base can be replaced with a modified base.
uauccacccaucc

SEQ ID NO: 391 - RNA, 13 nt, Artificial Sequence
  SEQ ID NO 391
  misc_feature (1)..(13): U can be replaced by T. Any base can be replaced with a modified base.
uuauccaaccauc

SEQ ID NO: 392 - RNA, 13 nt, Artificial Sequence
  SEQ ID NO 392
  misc_feature (1)..(13): U can be replaced by T. Any base can be replaced with a modified base.
uuauccacccauc

SEQ ID NO: 393 - RNA, 13 nt, Artificial Sequence
  SEQ ID NO 393
  misc_feature (1)..(13): U can be replaced by T. Any base can be replaced with a modified base.
uuuauccaaccau

SEQ ID NO: 394 - RNA, 13 nt, Artificial Sequence
  SEQ ID NO 394
  misc_feature (1)..(13): U can be replaced by T. Any base can be replaced with a modified base.
uuuauccacccau

SEQ ID NO: 395 - RNA, 13 nt, Artificial Sequence
  SEQ ID NO 395
  misc_feature (1)..(13): U can be replaced by T. Any base can be replaced with a modified base.
auuuauccaacca

SEQ ID NO: 396 - RNA, 13 nt, Artificial Sequence
  SEQ ID NO 396
  misc_feature (1)..(13): U can be replaced by T. Any base can be replaced with a modified base.
auuuauccaccca

SEQ ID NO: 397 - RNA, 13 nt, Artificial Sequence
  SEQ ID NO 397
  misc_feature (1)..(13): U can be replaced by T. Any base can be replaced with a modified base.
aauuuauccaacc

SEQ ID NO: 398 - RNA, 13 nt, Artificial Sequence
  SEQ ID NO 398
  misc_feature (1)..(13): U can be replaced by T. Any base can be replaced with a modified base.
aauuuauccaccc

SEQ ID NO: 399 - RNA, 13 nt, Artificial Sequence
  SEQ ID NO 399
  misc_feature (1)..(13): U can be replaced by T. Any base can be replaced with a modified base.
caauuuauccaac

SEQ ID NO: 400 - RNA, 13 nt, Artificial Sequence
  SEQ ID NO 400
  misc_feature (1)..(13): U can be replaced by T. Any base can be replaced with a modified base.
caauuuauccacc

SEQ ID NO: 401 - RNA, 13 nt, Artificial Sequence
  SEQ ID NO 401
  misc_feature (1)..(13): U can be replaced by T. Any base can be replaced with a modified base.
ucaauuuauccaa

SEQ ID NO: 402 - RNA, 13 nt, Artificial Sequence
  SEQ ID NO 402
  misc_feature (1)..(13): U can be replaced by T. Any base can be replaced with a modified base.
ucaauuuauccac

SEQ ID NO: 403 - RNA, 13 nt, Artificial Sequence
  SEQ ID NO 403
  misc_feature (1)..(13): U can be replaced by T. Any base can be replaced with a modified base.
aucaauuuaucca

SEQ ID NO: 404 - RNA, 13 nt, Artificial Sequence
  SEQ ID NO 404
  misc_feature (1)..(13): U can be replaced by T. Any base can be replaced with a modified base.
caucaauuuaucc

SEQ ID NO: 405 - RNA, 13 nt, Artificial Sequence
  SEQ ID NO 405
  misc_feature (1)..(13): U can be replaced by T. Any base can be replaced with a modified base.
ccaucaauuuauc

SEQ ID NO: 406 - RNA, 13 nt, Artificial Sequence
  SEQ ID NO 406
  misc_feature (1)..(13): U can be replaced by T. Any base can be replaced with a modified base.
cccaucaauuuau

SEQ ID NO: 407 - RNA, 13 nt, Artificial Sequence
  SEQ ID NO 407
  misc_feature (1)..(13): U can be replaced by T. Any base can be replaced with a modified base.
acccaucaauuua

SEQ ID NO: 408 - RNA, 13 nt, Artificial Sequence
  SEQ ID NO 408
  misc_feature (1)..(13): U can be replaced by T. Any base can be replaced with a modified base.
cacccaucaauuu

SEQ ID NO: 409 - RNA, 13 nt, Artificial Sequence
  SEQ ID NO 409
  misc_feature (1)..(13): U can be replaced by T. Any base can be replaced with a modified base.
ccacccaucaauu

SEQ ID NO: 410 - RNA, 13 nt, Artificial Sequence
  SEQ ID NO 410
  misc_feature (1)..(13): U can be replaced by T. Any base can be replaced with a modified base.
uccacccaucaau

SEQ ID NO: 411 - RNA, 13 nt, Artificial Sequence
  SEQ ID NO 411
  misc_feature (1)..(13): U can be replaced by T. Any base can be replaced with a modified base.
auccacccaucaa

SEQ ID NO: 412 - RNA, 13 nt, Artificial Sequence
  SEQ ID NO 412
  misc_feature (1)..(13): U can be replaced by T. Any base can be replaced with a modified base.
cauccacccauca

SEQ ID NO: 413 - RNA, 13 nt, Artificial Sequence
  SEQ ID NO 413
  misc_feature (1)..(13): U can be replaced by T. Any base can be replaced with a modified base.
ccauccacccauc

SEQ ID NO: 414 - RNA, 13 nt, Artificial Sequence
  SEQ ID NO 414
  misc_feature (1)..(13): U can be replaced by T. Any base can be replaced with a modified base.
uccauccacccau

SEQ ID NO: 415 - RNA, 13 nt, Artificial Sequence
  SEQ ID NO 415
  misc_feature (1)..(13): U can be replaced by T. Any base can be replaced with a modified base.
auccauccaccca

SEQ ID NO: 416 - RNA, 13 nt, Artificial Sequence
  SEQ ID NO 416
  misc_feature (1)..(13): U can be replaced by T. Any base can be replaced with a modified base.
cauccauccaccc

SEQ ID NO: 417 - RNA, 13 nt, Artificial Sequence
  SEQ ID NO 417
  misc_feature (1)..(13): U can be replaced by T. Any base can be replaced with a modified base.
ccauccauccacc

SEQ ID NO: 418 - RNA, 13 nt, Artificial Sequence
  SEQ ID NO 418
  misc_feature (1)..(13): U can be replaced by T. Any base can be replaced with a modified base.
accauccauccac

SEQ ID NO: 419 - RNA, 13 nt, Artificial Sequence
  SEQ ID NO 419
  misc_feature (1)..(13): U can be replaced by T. Any base can be replaced with a modified base.
aaccauccaucca

SEQ ID NO: 420 - RNA, 13 nt, Artificial Sequence
  SEQ ID NO 420
  misc_feature (1)..(13): U can be replaced by T. Any base can be replaced with a modified base.
caaccauccaucc

SEQ ID NO: 421 - RNA, 13 nt, Artificial Sequence
  SEQ ID NO 421
  misc_feature (1)..(13): U can be replaced by T. Any base can be replaced with a modified base.
ccaaccauccauc

SEQ ID NO: 422 - RNA, 13 nt, Artificial Sequence
  SEQ ID NO 422
  misc_feature (1)..(13): U can be replaced by T. Any base can be replaced with a modified base.
accaaccauccau

SEQ ID NO: 423 - RNA, 13 nt, Artificial Sequence
  SEQ ID NO 423
  misc_feature (1)..(13): U can be replaced by T. Any base can be replaced with a modified base.
aaccaaccaucca

SEQ ID NO: 424 - RNA, 13 nt, Artificial Sequence
  SEQ ID NO 424
  misc_feature (1)..(13): U can be replaced by T. Any base can be replaced with a modified base.
caaccaaccaucc

SEQ ID NO: 425 - RNA, 13 nt, Artificial Sequence
  SEQ ID NO 425
  misc_feature (1)..(13): U can be replaced by T. Any base can be replaced with a modified base.
acaaccaaccauc

SEQ ID NO: 426 - RNA, 13 nt, Artificial Sequence
  SEQ ID NO 426
  misc_feature (1)..(13): U can be replaced by T. Any base can be replaced with a modified base.
uacaaccaaccau

SEQ ID NO: 427 - RNA, 13 nt, Artificial Sequence
  SEQ ID NO 427
  misc_feature (1)..(13): U can be replaced by T. Any base can be replaced with a modified base.
uccgcaacuuaau

SEQ ID NO: 428 - RNA, 13 nt, Artificial Sequence
  SEQ ID NO 428
  misc_feature (1)..(13): U can be replaced by T. Any base can be replaced with a modified base.
auccgcaacuuaa

SEQ ID NO: 429 - RNA, 13 nt, Artificial Sequence
  SEQ ID NO 429
  misc_feature (1)..(13): U can be replaced by T. Any base can be replaced with a modified base.
gauccgcaacuua

SEQ ID NO: 430 - RNA, 13 nt, Artificial Sequence
  SEQ ID NO 430
  misc_feature (1)..(13): U can be replaced by T. Any base can be replaced with a modified base.
ugauccgcaacuu

SEQ ID NO: 431 - RNA, 13 nt, Artificial Sequence
  SEQ ID NO 431
  misc_feature (1)..(13): U can be replaced by T. Any base can be replaced with a modified base.
uugauccgcaacu

SEQ ID NO: 432 - RNA, 13 nt, Artificial Sequence
  SEQ ID NO 432
  misc_feature (1)..(13): U can be replaced by T. Any base can be replaced with a modified base.
auugauccgcaac

SEQ ID NO: 433 - RNA, 13 nt, Artificial Sequence
  SEQ ID NO 433
  misc_feature (1)..(13): U can be replaced by T. Any base can be replaced with a modified base.
cauugauccgcaa

SEQ ID NO: 434 - RNA, 13 nt, Artificial Sequence
  SEQ ID NO 434
  misc_feature (1)..(13)
acauugauccgca

SEQ ID NO: 435 - RNA, 13 nt, Artificial Sequence
  SEQ ID NO 435
  misc_feature (1)..(13): U can be replaced by T. Any base can be replaced with a modified base.
uacauugauccgc

SEQ ID NO: 436 - RNA, 13 nt, Artificial Sequence
  SEQ ID NO 436
  misc_feature (1)..(13): U can be replaced by T. Any base can be replaced with a modified base.
auacauugauccg

SEQ ID NO: 437 - RNA, 13 nt, Artificial Sequence
  SEQ ID NO 437
  misc_feature (1)..(13): U can be replaced by T. Any base can be replaced with a modified base.
cauacauugaucc

SEQ ID NO: 438 - RNA, 13 nt, Artificial Sequence
  SEQ ID NO 438
  misc_feature (1)..(13): U can be replaced by T. Any base can be replaced with a modified base.
ccauacauugauc

SEQ ID NO: 439 - RNA, 13 nt, Artificial Sequence
  SEQ ID NO 439
  misc_feature (1)..(13): U can be replaced by T. Any base can be replaced with a modified base.
cccauacauugau

SEQ ID NO: 440 - RNA, 13 nt, Artificial Sequence
  SEQ ID NO 440
  misc_feature (1)..(13): U can be replaced by T. Any base can be replaced with a modified base.
ucccauacauuga

SEQ ID NO: 441 - RNA, 13 nt, Artificial Sequence
  SEQ ID NO 441
  misc_feature (1)..(13): U can be replaced by T. Any base can be replaced with a modified base.
aucccauacauug

SEQ ID NO: 442 - RNA, 13 nt, Artificial Sequence
  SEQ ID NO 442
  misc_feature (1)..(13): U can be replaced by T. Any base can be replaced with a modified base.
caucccauacauu

SEQ ID NO: 443 - RNA, 13 nt, Artificial Sequence
  SEQ ID NO 443
  misc_feature (1)..(13): U can be replaced by T. Any base can be replaced with a modified base.
ccaucccauacau

SEQ ID NO: 444 - RNA, 13 nt, Artificial Sequence
  SEQ ID NO 444
  misc_feature (1)..(13): U can be replaced by T. Any base can be replaced with a modified base.
uccaucccauaca

SEQ ID NO: 445 - RNA, 13 nt, Artificial Sequence
  SEQ ID NO 445
  misc_feature (1)..(13): U can be replaced by T. Any base can be replaced with a modified base.
auccaucccauac

SEQ ID NO: 446 - RNA, 13 nt, Artificial Sequence
  SEQ ID NO 446
  misc_feature (1)..(13): U can be replaced by T. Any base can be replaced with a modified base.
cauccaucccaua

SEQ ID NO: 447 - RNA, 13 nt, Artificial Sequence
  SEQ ID NO 447
  misc_feature (1)..(13): U can be replaced by T. Any base can be replaced with a modified base.
ucauccaucccau

SEQ ID NO: 448 - RNA, 13 nt, Artificial Sequence
  SEQ ID NO 448
  misc_feature (1)..(13): U can be replaced by T. Any base can be replaced with a modified base.
uucauccauccca

SEQ ID NO: 449 - RNA, 13 nt, Artificial Sequence
  SEQ ID NO 449
  misc_feature (1)..(13): U can be replaced by T. Any base can be replaced with a modified base.
auucauccauccc

SEQ ID NO: 450 - RNA, 13 nt, Artificial Sequence
  SEQ ID NO 450
  misc_feature (1)..(13): U can be replaced by T. Any base can be replaced with a modified base.
cauucauccaucc

SEQ ID NO: 451 - RNA, 13 nt, Artificial Sequence
  SEQ ID NO 451
  misc_feature (1)..(13): U can be replaced by T. Any base can be replaced with a modified base.
ccauucauccauc

SEQ ID NO: 452 - RNA, 13 nt, Artificial Sequence
  SEQ ID NO 452
  misc_feature (1)..(13): U can be replaced by T. Any base can be replaced with a modified base.
uccauucauccau

SEQ ID NO: 453 - RNA, 13 nt, Artificial Sequence
  SEQ ID NO 453
  misc_feature (1)..(13): U can be replaced by T. Any base can be replaced with a modified base.
auccauucaucca

SEQ ID NO: 454 - RNA, 12 nt, Artificial Sequence
  SEQ ID NO 454
  misc_feature (1)..(13): U can be replaced by T. Any base can be replaced with a modified base.
cauccauucauc

SEQ ID NO: 455 - RNA, 13 nt, Artificial Sequence
  SEQ ID NO 455
  misc_feature (1)..(13): U can be replaced by T. Any base can be replaced with a modified base.
ccauccauucauc

SEQ ID NO: 456 - RNA, 13 nt, Artificial Sequence
  SEQ ID NO 456
  misc_feature (1)..(13): U can be replaced by T. Any base can be replaced with a modified base.
uccauccauucau

SEQ ID NO: 457 - RNA, 13 nt, Artificial Sequence
  SEQ ID NO 457
  misc_feature (1)..(13): U can be replaced by T. Any base can be replaced with a modified base.
auccauccauuca

SEQ ID NO: 458 - RNA, 13 nt, Artificial Sequence
  SEQ ID NO 458
  misc_feature (1)..(13): U can be replaced by T. Any base can be replaced with a modified base.
cauccauccauuc

SEQ ID NO: 459 - RNA, 13 nt, Artificial Sequence
  SEQ ID NO 459
  misc_feature (1)..(13): U can be replaced by T. Any base can be replaced with a modified base.
ccauccauccauu

SEQ ID NO: 460 - RNA, 13 nt, Artificial Sequence
  SEQ ID NO 460
  misc_feature (1)..(13): U can be replaced by T. Any base can be replaced with a modified base.
uccauccauccau

SEQ ID NO: 461 - RNA, 13 nt, Artificial Sequence
  SEQ ID NO 461
  misc_feature (1)..(13): U can be replaced by T. Any base can be replaced with a modified base.
auccauccaucca

SEQ ID NO: 462 - RNA, 13 nt, Artificial Sequence
  SEQ ID NO 462
  misc_feature (1)..(13): U can be replaced by T. Any base can be replaced with a modified base.
cauccauccaucc

SEQ ID NO: 463 - RNA, 13 nt, Artificial Sequence
  SEQ ID NO 463
  misc_feature (1)..(13): U can be replaced by T. Any base can be replaced with a modified base.
ccauccauccauc

SEQ ID NO: 464 - RNA, 13 nt, Artificial Sequence
  SEQ ID NO 464
  misc_feature (1)..(13): U can be replaced by T. Any base can be replaced with a modified base.
acauccauccauc

SEQ ID NO: 465 - RNA, 13 nt, Artificial Sequence
  SEQ ID NO 465
  misc_feature (1)..(13): U can be replaced by T. Any base can be replaced with a modified base.
cacauccauccau

SEQ ID NO: 466 - RNA, 13 nt, Artificial Sequence
  SEQ ID NO 466
  misc_feature (1)..(13): U can be replaced by T. Any base can be replaced with a modified base.
acacauccaucca

SEQ ID NO: 467 - RNA, 13 nt, Artificial Sequence
  SEQ ID NO 467
  misc_feature (1)..(13): U can be replaced by T. Any base can be replaced with a modified base.
cacacauccaucc

SEQ ID NO: 468 - RNA, 13 nt, Artificial Sequence
  SEQ ID NO 468
  misc_feature (1)..(13): U can be replaced by T. Any base can be replaced with a modified base.
ccacacauccauc

SEQ ID NO: 469 - RNA, 13 nt, Artificial Sequence
  SEQ ID NO 469
  misc_feature (1)..(13): U can be replaced by T. Any base can be replaced with a modified base.
accacacauccau

SEQ ID NO: 470 - RNA, 13 nt, Artificial Sequence
  SEQ ID NO 470
  misc_feature (1)..(13): U can be replaced by T. Any base can be replaced with a modified base.
aaccacacaucca

SEQ ID NO: 471 - RNA, 13 nt, Artificial Sequence
  SEQ ID NO 471
  misc_feature (1)..(13): U can be replaced by T. Any base can be replaced with a modified base.
caaccacacaucc

SEQ ID NO: 472 - RNA, 13 nt, Artificial Sequence
  SEQ ID NO 472
  misc_feature (1)..(13): U can be replaced by T. Any base can be replaced with a modified base.
ucaaccacacauc

SEQ ID NO: 473 - RNA, 13 nt, Artificial Sequence
  SEQ ID NO 473
  misc_feature (1)..(13): U can be replaced by T. Any base can be replaced with a modified base.
uucaaccacacau

SEQ ID NO: 474 - RNA, 13 nt, Artificial Sequence
  SEQ ID NO 474
  misc_feature (1)..(13): U can be replaced by T. Any base can be replaced with a modified base.
auucaaccacaca

SEQ ID NO: 475 - RNA, 13 nt, Artificial Sequence
  SEQ ID NO 475
  misc_feature (1)..(13): U can be replaced by T. Any base can be replaced with a modified base.
ucuauccagcaau

SEQ ID NO: 476 - RNA, 13 nt, Artificial Sequence
  SEQ ID NO 476
  misc_feature (1)..(13): U can be replaced by T. Any base can be replaced with a modified base.
aucuauccagcaa

SEQ ID NO: 477 - RNA, 13 nt, Artificial Sequence
  SEQ ID NO 477
  misc_feature (1)..(13): U can be replaced by T. Any base can be replaced with a modified base.
caucuauccagca

SEQ ID NO: 478 - RNA, 13 nt, Artificial Sequence
  SEQ ID NO 478
  misc_feature (1)..(13): U can be replaced by T. Any base can be replaced with a modified base.
ucaucuauccagc

SEQ ID NO: 479 - RNA, 13 nt, Artificial Sequence
  SEQ ID NO 479
  misc_feature (1)..(13): U can be replaced by T. Any base can be replaced with a modified base.
aucaucuauccag

SEQ ID NO: 480 - RNA, 13 nt, Artificial Sequence
  SEQ ID NO 480
  misc_feature (1)..(13): U can be replaced by T. Any base can be replaced with a modified base.
aaucaucuaucca

SEQ ID NO: 481 - RNA, 13 nt, Artificial Sequence
  SEQ ID NO 481
  misc_feature (1)..(13): U can be replaced by T. Any base can be replaced with a modified base.
caaucaucuaucc

SEQ ID NO: 482 - RNA, 13 nt, Artificial Sequence
  SEQ ID NO 482
  misc_feature (1)..(13): U can be replaced by T. Any base can be replaced with a modified base.
ucaaucaucuauc

SEQ ID NO: 483 - RNA, 13 nt, Artificial Sequence
  SEQ ID NO 483
  misc_feature (1)..(13): U can be replaced by T. Any base can be replaced with a modified base.
gucaaucaucuau

SEQ ID NO: 484 - RNA, 13 nt, Artificial Sequence
  SEQ ID NO 484
  misc_feature (1)..(13): U can be replaced by T. Any base can be replaced with a modified base.
agucaaucaucua

SEQ ID NO: 485 - RNA, 13 nt, Artificial Sequence
  SEQ ID NO 485
  misc_feature (1)..(13): U can be replaced by T. Any base can be replaced with a modified base.
cagucaaucaucu

SEQ ID NO: 486 - RNA, 13 nt, Artificial Sequence
  SEQ ID NO 486
  misc_feature (1)..(13): U can be replaced by T. Any base can be replaced with a modified base.
ccagucaaucauc

SEQ ID NO: 487 - RNA, 13 nt, Artificial Sequence
  SEQ ID NO 487
  misc_feature (1)..(13): U can be replaced by T. Any base can be replaced with a modified base.
cccagucaaucau

SEQ ID NO: 488 - RNA, 13 nt, Artificial Sequence
  SEQ ID NO 488
  misc_feature (1)..(13): U can be replaced by T. Any base can be replaced with a modified base.
acccagucaauca

SEQ ID NO: 489 - RNA, 13 nt, Artificial Sequence
  SEQ ID NO 489
  misc_feature (1)..(13): U can be replaced by T. Any base can be replaced with a modified base.
cacccagucaauc

SEQ ID NO: 490 - RNA, 13 nt, Artificial Sequence
  SEQ ID NO 490
  misc_feature (1)..(13): U can be replaced by T. Any base can be replaced with a modified base.
ccacccagucaau

SEQ ID NO: 491 - RNA, 13 nt, Artificial Sequence
  SEQ ID NO 491
  misc_feature (1)..(13): U can be replaced by T. Any base can be replaced with a modified base.
uccacccagucaa

SEQ ID NO: 492 - RNA, 13 nt, Artificial Sequence
  SEQ ID NO 492
  misc_feature (1)..(13): U can be replaced by T. Any base can be replaced with a modified base.
auccacccaguca

SEQ ID NO: 493 - RNA, 13 nt, Artificial Sequence
  SEQ ID NO 493
  misc_feature (1)..(13): U can be replaced by T. Any base can be replaced with a modified base.
uauccacccaguc

SEQ ID NO: 494 - RNA, 13 nt, Artificial Sequence
  SEQ ID NO 494
  misc_feature (1)..(13): U can be replaced by T. Any base can be replaced with a modified base.
cuauccacccagu

SEQ ID NO: 495 - RNA, 13 nt, Artificial Sequence
  SEQ ID NO 495
  misc_feature (1)..(13): U can be replaced by T. Any base can be replaced with a modified base.
ucuauccacccag

SEQ ID NO: 496 - RNA, 13 nt, Artificial Sequence
  SEQ ID NO 496
  misc_feature (1)..(13): U can be replaced by T. Any base can be replaced with a modified base.
aucuauccaccca

SEQ ID NO: 497 - RNA, 13 nt, Artificial Sequence
  SEQ ID NO 497
  misc_feature (1)..(13): U can be replaced by T. Any base can be replaced with a modified base.
caucuauccaccc

SEQ ID NO: 498 - RNA, 13 nt, Artificial Sequence
  SEQ ID NO 498
  misc_feature (1)..(13): U can be replaced by T. Any base can be replaced with a modified base.
ucaucuauccacc

SEQ ID NO: 499 - RNA, 13 nt, Artificial Sequence
  SEQ ID NO 499
  misc_feature (1)..(13): U can be replaced by T. Any base can be replaced with a modified base.
uucaucuauccac

SEQ ID NO: 500 - RNA, 13 nt, Artificial Sequence
  SEQ ID NO 500
  misc_feature (1)..(13): U can be replaced by T. Any base can be replaced with a modified base.
uuucaucuaucca

SEQ ID NO: 501 - RNA, 13 nt, Artificial Sequence
  SEQ ID NO 501
auuucaucuaucc

SEQ ID NO: 502 - RNA, 13 nt, Artificial Sequence
  SEQ ID NO 502
  misc_feature (1)..(13): U can be replaced by T. Any base can be replaced with a modified base.
cauuucaucuauc

SEQ ID NO: 503 - RNA, 13 nt, Artificial Sequence
  SEQ ID NO 503
  misc_feature (1)..(13): U can be replaced by T. Any base can be replaced with a modified base.
acauuucaucuau

SEQ ID NO: 504 - RNA, 13 nt, Artificial Sequence
  SEQ ID NO 504
  misc_feature (1)..(13): U can be replaced by T. Any base can be replaced with a modified base.
aacauuucaucua

SEQ ID NO: 505 - RNA, 13 nt, Artificial Sequence
  SEQ ID NO 505
  misc_feature (1)..(13): U can be replaced by T. Any base can be replaced with a modified base.
caacauuucaucu

SEQ ID NO: 506 - RNA, 13 nt, Artificial Sequence
  SEQ ID NO 506
  misc_feature (1)..(13): U can be replaced by T. Any base can be replaced with a modified base.
ucuggggcagcuu

SEQ ID NO: 507 - RNA, 13 nt, Artificial Sequence
  SEQ ID NO 507
  misc_feature (1)..(13): U can be replaced by T. Any base can be replaced with a modified base.
gucuggggcagcu

SEQ ID NO: 508 - RNA, 13 nt, Artificial Sequence
  SEQ ID NO 508
  misc_feature (1)..(13): U can be replaced by T. Any base can be replaced with a modified base.
ggucuggggcagc

SEQ ID NO: 509 - RNA, 13 nt, Artificial Sequence
  SEQ ID NO 509
  misc_feature (1)..(13): U can be replaced by T. Any base can be replaced with a modified base.
gggucuggggcag

SEQ ID NO: 510 - RNA, 13 nt, Artificial Sequence
  SEQ ID NO 510
  misc_feature (1)..(13): U can be replaced by T. Any base can be replaced with a modified base.
agggucuggggca

SEQ ID NO: 511 - RNA, 13 nt, Artificial Sequence
  SEQ ID NO 511
  misc_feature (1)..(13): U can be replaced by T. Any base can be replaced with a modified base.
cagggucuggggc

SEQ ID NO: 512 - RNA, 13 nt, Artificial Sequence
  SEQ ID NO 512
  misc_feature (1)..(13): U can be replaced by T. Any base can be replaced with a modified base.
ccagggucugggg

SEQ ID NO: 513 - RNA, 13 nt, Artificial Sequence
  SEQ ID NO 513
  misc_feature (1)..(13): U can be replaced by T. Any base can be replaced with a modified base.
cccagggucuggg

SEQ ID NO: 514 - RNA, 13 nt, Artificial Sequence
  SEQ ID NO 514
  misc_feature (1)..(13): U can be replaced by T. Any base can be replaced with a modified base.
ucccagggucugg

SEQ ID NO: 515 - RNA, 13 nt, Artificial Sequence
  SEQ ID NO 515
  misc_feature (1)..(13): U can be replaced by T. Any base can be replaced with a modified base.
gucccagggucug

SEQ ID NO: 516 - RNA, 13 nt, Artificial Sequence
  SEQ ID NO 516
  misc_feature (1)..(13): U can be replaced by T. Any base can be replaced with a modified base.
ggucccagggucu

SEQ ID NO: 517 - RNA, 13 nt, Artificial Sequence
  SEQ ID NO 517
  misc_feature (1)..(13): U can be replaced by T. Any base can be replaced with a modified base.
aggucccaggguc

SEQ ID NO: 518 - RNA, 13 nt, Artificial Sequence
  SEQ ID NO 518
  misc_feature (1)..(13): U can be replaced by T. Any base can be replaced with a modified base.
gaggucccagggu

SEQ ID NO: 519 - RNA, 13 nt, Artificial Sequence
  SEQ ID NO 519
  misc_feature (1)..(13): U can be replaced by T. Any base can be replaced with a modified base.
agaggucccaggg

SEQ ID NO: 520 - RNA, 13 nt, Artificial Sequence
  SEQ ID NO 520
  misc_feature (1)..(13): U can be replaced by T. Any base can be replaced with a modified base.
cagaggucccagg

SEQ ID NO: 521 - RNA, 13 nt, Artificial Sequence
  SEQ ID NO 521
  misc_feature (1)..(13): U can be replaced by T. Any base can be replaced with a modified base.
ucagaggucccag

SEQ ID NO: 522 - RNA, 13 nt, Artificial Sequence
  SEQ ID NO 522
  misc_feature (1)..(13): U can be replaced by T. Any base can be replaced with a modified base.
gucagagguccca

SEQ ID NO: 523 - RNA, 13 nt, Artificial Sequence
  SEQ ID NO 523
  misc_feature (1)..(13): U can be replaced by T. Any base can be replaced with a modified base.
ggucagagguccc

SEQ ID NO: 524 - RNA, 13 nt, Artificial Sequence
  SEQ ID NO 524
  misc_feature (1)..(13): U can be replaced by T. Any base can be replaced with a modified base.
gggucagaggucc

SEQ ID NO: 525 - RNA, 13 nt, Artificial Sequence
  SEQ ID NO 525
  misc_feature (1)..(13): U can be replaced by T. Any base can be replaced with a modified base.
ggggucagagguc

SEQ ID NO: 526 - RNA, 13 nt, Artificial Sequence
  SEQ ID NO 526
  misc_feature (1)..(13): U can be replaced by T. Any base can be replaced with a modified base.
gggggucagaggu

SEQ ID NO: 527 - RNA, 13 nt, Artificial Sequence
  SEQ ID NO 527
  misc_feature (1)..(13): U can be replaced by T. Any base can be replaced with a modified base.
cgggggucagagg

SEQ ID NO: 528 - RNA, 13 nt, Artificial Sequence
  SEQ ID NO 528
  misc_feature (1)..(13): U can be replaced by T. Any base can be replaced with a modified base.
ccgggggucagag

SEQ ID NO: 529 - RNA, 13 nt, Artificial Sequence
  SEQ ID NO 529
  misc_feature (1)..(13): U can be replaced by T. Any base can be replaced with a modified base.
gccgggggucaga

SEQ ID NO: 530 - RNA, 13 nt, Artificial Sequence
  SEQ ID NO 530
  misc_feature (1)..(13): U can be replaced by T. Any base can be replaced with a modified base.
cgccgggggucag

SEQ ID NO: 531 - RNA, 13 nt, Artificial Sequence
  SEQ ID NO 531
  misc_feature (1)..(13): U can be replaced by T. Any base can be replaced with a modified base.
ucgccggggguca

SEQ ID NO: 532 - RNA, 13 nt, Artificial Sequence
  SEQ ID NO 532
  misc_feature (1)..(13): U can be replaced by T. Any base can be replaced with a modified base.
gucgccggggguc

SEQ ID NO: 533 - RNA, 13 nt, Artificial Sequence
  SEQ ID NO 534
  misc_feature (1)..(13): U can be replaced by T. Any base can be replaced with a modified base.
ggucgccgggggu

SEQ ID NO: 534 - RNA, 13 nt, Artificial Sequence
  SEQ ID NO 534
  misc_feature (1)..(13): U can be replaced by T. Any base can be replaced with a modified base.
gggucgccggggg

SEQ ID NO: 535 - RNA, 13 nt, Artificial Sequence
  SEQ ID NO 535
  misc_feature (1)..(13): U can be replaced by T. Any base can be replaced with a modified base.
ggggucgccgggg

SEQ ID NO: 536 - RNA, 13 nt, Artificial Sequence
  SEQ ID NO 536
  misc_feature (1)..(13): U can be replaced by T. Any base can be replaced with a modified base.
aggggucgccggg

SEQ ID NO: 537 - RNA, 13 nt, Artificial Sequence
  SEQ ID NO 537
  misc_feature (1)..(13): U can be replaced by T. Any base can be replaced with a modified base.
aaggggucgccgg

SEQ ID NO: 538 - RNA, 13 nt, Artificial Sequence
  SEQ ID NO 538
  misc_feature (1)..(13): U can be replaced by T. Any base can be replaced with a modified base.
caaggggucgccg

SEQ ID NO: 539 - RNA, 13 nt, Artificial Sequence
  SEQ ID NO 539
  misc_feature (1)..(13): U can be replaced by T. Any base can be replaced with a modified base.
gcaaggggucgcc

SEQ ID NO: 540 - RNA, 13 nt, Artificial Sequence
  SEQ ID NO 540
  misc_feature (1)..(13): U can be replaced by T. Any base can be replaced with a modified base.
ugcaaggggucgc

SEQ ID NO: 541 - RNA, 13 nt, Artificial Sequence
  SEQ ID NO 541
  misc_feature (1)..(13): U can be replaced by T. Any base can be replaced with a modified base.
gugcaaggggucg

SEQ ID NO: 542 - RNA, 13 nt, Artificial Sequence
  SEQ ID NO 542
  misc_feature (1)..(13): U can be replaced by T. Any base can be replaced with a modified base.
agugcaagggguc

SEQ ID NO: 543 - RNA, 13 nt, Artificial Sequence
  SEQ ID NO 545
  misc_feature (1)..(13): U can be replaced by T. Any base can be replaced with a modified base.
gagugcaaggggu

SEQ ID NO: 544 - RNA, 13 nt, Artificial Sequence
  SEQ ID NO 544
  misc_feature (1)..(13): U can be replaced by T. Any base can be replaced with a modified base.
agagugcaagggg

SEQ ID NO: 545 - RNA, 13 nt, Artificial Sequence
  SEQ ID NO 545
  misc_feature (1)..(13): U can be replaced by T. Any base can be replaced with a modified base.
gagagugcaaggg

SEQ ID NO: 546 - RNA, 13 nt, Artificial Sequence
  SEQ ID NO 546
  misc_feature (1)..(13): U can be replaced by T. Any base can be replaced with a modified base.
ggagagugcaagg

SEQ ID NO: 547 - RNA, 80 nt, Homo sapiens
augaguagauaaaaggauggauggagagaugggugaguacauggauggauagauggaugaguugguggguagauucgugc

SEQ ID NO: 548 - RNA, 80 nt, Homo sapiens
augaguagauaaaagcauggauggagagaugggugaguacauggauggauagauggaugaguugguggguagauucgugc

SEQ ID NO: 549 - RNA, 40 nt, Homo sapiens
ggauggauggagagaugggugaguacauggauggauagau

SEQ ID NO: 550 - RNA, 40 nt, Homo sapiens
gcauggauggagagaugggugaguacauggauggauagau

SEQ ID NO: 551 - RNA, 29 nt, Homo sapiens
auggagagaugggugaguacauggaugga

SEQ ID NO: 552 - RNA, 97 nt, Homo sapiens
guucuuccuucuauuccagcccuaaccacucaggauugggccguuugugucuggguaugucucuuccagcugccuggguuuccuggaaagaacucuu

SEQ ID NO: 553 - RNA, 43 nt, Homo sapiens
gugucuggguaugucucuuccagcugccuggguuuccuggaaa

SEQ ID NO: 554 - RNA, 46 nt, Homo sapiens
ucaucagguucuuccuucuauuccagcccuaaccacucaggauugg

SEQ ID NO: 555 - DNA, 21 bp, Artificial Sequence
  21nt_SNP&DonMix1
  modified_base (1)..(21): * = a phosphorothioate, + = LNA
  modified_base (1)..(21): phosphorothioate linkage, LNA at positions 1, 4, 7, 10, 13, 16, 19
cacccatctctccatccatgc

SEQ ID NO: 556 - DNA, 21 bp, Artificial Sequence
  21nt_SNP&DonMix2
  modified_base (1)..(21): phosphorthioate backbone, and LNA at positions 1, 4, 7, 10, 13, 16 and 19
  modified_base (1)..(21): phosphorthioate linkage, and LNA at positions 1, 4, 7, 10, 13, 16 and 19
cacccatctctccatccatcc

SEQ ID NO: 557 - DNA, 21 bp, Artificial Sequence
  21nt_Don1
  modified_base (1)..(21): phosphorthioate backbone, LNA at positions 1, 4, 7, 10, 13, 16, 19 and 21
  modified_base (1)..(21): phosphorthioate linkage, LNA at positions 1, 4, 7, 10, 13, 16, 19 and 21
ctcacccatctctccatccat

SEQ ID NO: 558 - DNA, 21 bp, Artificial Sequence
  21nt_Don2
  modified_base (1)..(21): phosphorthioate backbone, LNA at positions 1, 4, 7, 10, 13, 16, 19 and 21
  modified_base (1)..(21): phosphorthioate linkage, LNA at positions 1, 4, 7, 10, 13, 16, 19 and 21
tgtactcacccatctctccat

SEQ ID NO: 559 - DNA, 21 bp, Artificial Sequence
  21nt_Don3
  modified_base (1)..(21): phosphorthioate backbone, LNA at positions 1, 4, 7, 10, 13, 16, 19 and 21
  modified_base (1)..(21): phosphorthioate linkage, LNA at positions 1, 4, 7, 10, 13, 16, 19 and 21
tccatgtactcacccatctct

SEQ ID NO: 560 - DNA, 21 bp, Artificial Sequence
  21nt_Don4
  modified_base (1)..(21): phosphorthioate backbone, LNA at positions 1, 4, 7, 10, 13, 16, 19 and 21
  modified_base (1)..(21): phosphorthioate linkage, LNA at positions 1, 4, 7, 10, 13, 16, 19 and 21
tccatccatgtactcacccat

SEQ ID NO: 561 - DNA, 21 bp, Artificial Sequence
  21nt_Don5
  modified_base (1)..(21): phosphorthioate backbone, LNA at positions 1, 4, 7, 10, 13, 16, 19 and 21
  modified_base (1)..(21): phosphorthioate linkage, LNA at positions 1, 4, 7, 10, 13, 16, 19 and 21
atctatccatccatgtactca

SEQ ID NO: 562 - DNA, 17 bp, Artificial Sequence
  17nt_Don1
  modified_base (1)..(17): phosphorthioate backbone, LNA at postions 1, 4, 7, 10, 13, 16 and 17
  modified_base (1)..(17): phosphorthioate linkage, LNA at postions 1, 4, 7, 10, 13, 16 and 17
tcacccatctctccatc

SEQ ID NO: 563 - DNA, 17 bp, Artificial Sequence
  17nt_Don2
  modified_base (1)..(17): phosphorothioate linkage, LNA at 1, 3, 5, 7, 9, 11, 13, 15 and 17
tcacccatctctccatc

SEQ ID NO: 564 - DNA, 17 bp, Artificial Sequence
  17nt_Don3
  modified_base (1)..(17): phosphorthioate backbone, LNA bases at 1, 4, 7, 10, 13, 16 and 17
  modified_base (1)..(17): phosphorothioate linkage, LNA bases at 1, 4, 7, 10, 13, 16 and 17
gtactcacccatctctc

SEQ ID NO: 565 - DNA, 17 bp, Artificial Sequence
  17nt_Don4
  modified_base (1)..(17): phosphorthioate backbone, LNA at positins 1, 3, 5, 7, 9, 11, 13, 15 and 17
gtactcacccatctctc

SEQ ID NO: 566 - DNA, 13 bp, Artificial Sequence
  13nt_Don1
  modified_base (1)..(13): phosphorthioate backbone, LNA bases at 2, 4, 6, 8, 10 and 12
  modified_base (1)..(13): phosphorthioate linkage, LNA bases at 2, 4, 6, 8, 10 and 12
cacccatctctcc

SEQ ID NO: 567 - RNA, 25 nt, Artificial Sequence
  OMe_25nt_Don
  modified_base (1)..(25): phosphorthioate backbone and 2-OMe-RNA at all positions
  modified_base (1)..(25): phosphorthioate linkage and 2-OMe-RNA at all positions
cauguacucacccaucucuccaucc

SEQ ID NO: 568 - RNA, 30 nt, Artificial Sequence
  OMe_30nt_Don
  modified_base (1)..(30): phosphorthioate backbone, all bases substitued with 2--O-methyl-RNA
  modified_base (1)..(30): phosphorthioate linkage, all bases substitued with 2--O-methyl-RNA
auccauguacucacccaucucuccauccau

SEQ ID NO: 569 - DNA, 21 bp, Artificial Sequence
  21nt_ShortAcc2
  modified_base (1)..(21): phosphorthioate backbone, LNA at positions 1, 4, 7, 10, 13, 16, 19 and 21
  modified_base (1)..(21): phosphorthioate linkage, LNA at positions 1, 4, 7, 10, 13, 16, 19 and 21
caggcagctggaagagacata

SEQ ID NO: 570 - DNA, 21 bp, Artificial Sequence
  21nt_Short Acc3
  modified_base (1)..(21): phosphorothioate linkage, LNA  at positions 2, 4, 7, 10, 13, 16, 19 and 21
aacccaggcagctggaagaga

SEQ ID NO: 571 - DNA, 21 bp, Artificial Sequence
  21nt_ShortAcc4
  modified_base (1)..(21): phosphorthioate backbone, LNA at positions 1, 4, 7, 10, 13, 16, 19 and 21
  modified_base (1)..(21): phosphorthioate linkage, LNA at positions 1, 4, 7, 10, 13, 16, 19 and 21
ggaaacccaggcagctggaag

SEQ ID NO: 572 - DNA, 13 bp, Artificial Sequence
  Scrambled Control
agttttcaattcc

SEQ ID NO: 573 - DNA, 20 bp, Artificial Sequence
  Nest1_F
gacatcaaatcccgcgtgaa

SEQ ID NO: 574 - DNA, 20 bp, Artificial Sequence
  Nest1_R
cattgatgttggcgagcagg

SEQ ID NO: 575 - DNA, 20 bp, Artificial Sequence
  Nest2_F
cagacgatcattgaggtgcg

SEQ ID NO: 576 - DNA, 20 bp, Artificial Sequence
  SEQ ID NO 575
atacttggaggagaggcagg

SEQ ID NO: 577 - DNA, 18 bp, Artificial Sequence
  Single_F
caagcgaactgacaaatc

SEQ ID NO: 578 - DNA, 17 bp, Artificial Sequence
  Single_R
ctgggatcttcacgacc

SEQ ID NO: 579 - DNA, 21 bp, Artificial Sequence
  21nt_LongAcc1
  modified_base (1)..(21): phosphorothioate linkage, LNA at bases 1, 4, 7, 10, 13, 16, 19, and 21
tagggctggaatagaaggaag

SEQ ID NO: 580 - DNA, 21 bp, Artificial Sequence
  21nt_LongAcc2
  modified_base (1)..(21): phosphorothioate linkage, LNA at bases 1, 4, 7, 10, 13, 16, 19, and 21
tgagtggttagggctggaata